European Patent Specification EP 3 560 959 B1, published November 22, 2023. Title: ANTIBODY MOLECULES TO TIM-3 AND USES THEREOF. Applicant: NOVARTIS AG DANA-FARBER CANCER INSTITUTE, INC. CHILDREN'S MEDICAL CENTER CORPORATION. The sequence listing filed with the application follows.

SEQUENCE LISTING (142 sequences)

SEQ ID NO: 1 - protein, 118 aa, Artificial Sequence
  source: /note="Description of Artificial Sequence: Synthetic polypeptide"
QVQLQQPGAELVKPGASVKMSCKASGYTFTSYNMHWIKQTPGQGLEWIGDIYPGNGDTSYNQKFKGKATLTADKSSSTVYMQLSSLTSEDSAVYYCARVGGAFPMDYWGQGTSVTVSS

SEQ ID NO: 2 - protein, 111 aa, Artificial Sequence
  source: /note="Description of Artificial Sequence: Synthetic polypeptide"
DIVLTQSPASLAVSLGQRATISCRASESVEYYGTSLMQWYQQKPGQPPKLLIYAASNVESGVPARFSGSGSGTDFSLNIHPVEEDDIAIYFCQQSRKDPSTFGGGTKLEIK

SEQ ID NO: 3 - protein, 5 aa, Artificial Sequence
  source: /note="Description of Artificial Sequence: Synthetic peptide"
SYNMH

SEQ ID NO: 4 - protein, 17 aa, Artificial Sequence
  source: /note="Description of Artificial Sequence: Synthetic peptide"
DIYPGNGDTSYNQKFKG

SEQ ID NO: 5 - protein, 9 aa, Artificial Sequence
  source: /note="Description of Artificial Sequence: Synthetic peptide"
VGGAFPMDY

SEQ ID NO: 6 - protein, 15 aa, Artificial Sequence
  source: /note="Description of Artificial Sequence: Synthetic peptide"
RASESVEYYGTSLMQ

SEQ ID NO: 7 - protein, 7 aa, Artificial Sequence
  source: /note="Description of Artificial Sequence: Synthetic peptide"
AASNVES

SEQ ID NO: 8 - protein, 9 aa, Artificial Sequence
  source: /note="Description of Artificial Sequence: Synthetic peptide"
QQSRKDPST

SEQ ID NO: 9 - protein, 7 aa, Artificial Sequence
  source: /note="Description of Artificial Sequence: Synthetic peptide"
GYTFTSY

SEQ ID NO: 10 - protein, 6 aa, Artificial Sequence
  source: /note="Description of Artificial Sequence: Synthetic peptide"
YPGNGD

SEQ ID NO: 11 - DNA, 354 bp, Artificial Sequence
  Description of Artificial Sequence: Synthetic polynucleotide
caggtgcaactgcagcagcctggggctgagctggtgaagcctggggcctcagtgaagatgtcctgcaaggcttctggctacacatttaccagttacaatatgcactggataaagcagacacctggacagggcctggaatggattggagatatttatccaggaaatggtgatacttcctacaatcagaaattcaaaggcaaggccacattgactgcagacaaatcctccagcacagtctacatgcagctcagcagcctgacatctgaggactctgcggtctattactgtgcaagagtggggggtgcctttcctatggactactggggtcaaggaacctcagtcaccgtctcctca

SEQ ID NO: 12 - protein, 11 aa, Artificial Sequence
  source: /note="Description of Artificial Sequence: Synthetic peptide"
SESVEYYGTSL

SEQ ID NO: 13 - protein, 3 aa, Artificial Sequence
  source: /note="Description of Artificial Sequence: Synthetic peptide"
AAS

SEQ ID NO: 14 - protein, 6 aa, Artificial Sequence
  source: /note="Description of Artificial Sequence: Synthetic peptide"
SRKDPS

SEQ ID NO: 15 - DNA, 333 bp, Artificial Sequence
  source: /note="Description of Artificial Sequence: Synthetic polynucleotide"
gacattgtgctcacccaatctccagcttctttggctgtgtctctagggcagagagccaccatctcctgcagagccagtgaaagtgttgaatattatggcacaagtttaatgcagtggtaccaacagaaaccaggacagccacccaaactcctcatctatgctgcatccaacgtagaatctggggtccctgccaggtttagtggcagtgggtctgggacagacttcagcctcaacatccatcctgtggaggaggatgatattgcaatatatttctgtcagcaaagtaggaaggatccttcgacgttcggtggaggcaccaagctggagatcaaa

SEQ ID NO: 16 - protein, 118 aa, Artificial Sequence
  source: /note="Description of Artificial Sequence: Synthetic polypeptide"
QVQLVQSGAEVKKPGASVKVSCKASGYTFTSYNMHWVRQAPGQGLEWIGDIYPGNGDTSYNQKFKGRATMTADKSTSTVYMELSSLRSEDTAVYYCARVGGAFPMDYWGQGTLVTVSS

SEQ ID NO: 17 - DNA, 354 bp, Artificial Sequence
  source: /note="Description of Artificial Sequence: Synthetic polynucleotide"
caggtgcagctggtgcagtcaggcgccgaagtgaagaaacccggcgctagtgtgaaagtctcttgtaaagctagtggctacaccttcactagctataatatgcactgggttcgccaggccccagggcagggcctcgagtggatcggcgatatctaccccgggaacggcgacactagttataatcagaagtttaagggtagagctactatgaccgccgataagtctactagcaccgtctatatggaactgagttccctgaggtctgaggacaccgccgtctactactgcgctagagtgggcggagccttccctatggactactggggtcaaggcaccctggtcaccgtgtctagc

SEQ ID NO: 18 - protein, 444 aa, Artificial Sequence
  source: /note="Description of Artificial Sequence: Synthetic polypeptide"
QVQLVQSGAEVKKPGASVKVSCKASGYTFTSYNMHWVRQAPGQGLEWIGDIYPGNGDTSYNQKFKGRATMTADKSTSTVYMELSSLRSEDTAVYYCARVGGAFPMDYWGQGTLVTVSSASTKGPSVFPLAPCSRSTSESTAALGCLVKDYFPEPVTVSWNSGALTSGVHTFPAVLQSSGLYSLSSVVTVPSSSLGTKTYTCNVDHKPSNTKVDKRVESKYGPPCPPCPAPEFLGGPSVFLFPPKPKDTLMISRTPEVTCVVVDVSQEDPEVQFNWYVDGVEVHNAKTKPREEQFNSTYRVVSVLTVLHQDWLNGKEYKCKVSNKGLPSSIEKTISKAKGQPREPQVYTLPPSQEEMTKNQVSLTCLVKGFYPSDIAVEWESNGQPENNYKTTPPVLDSDGSFFLYSRLTVDKSRWQEGNVFSCSVMHEALHNHYTQKSLSLSLG

SEQ ID NO: 19 - DNA, 1332 bp, Artificial Sequence
  source: /note="Description of Artificial Sequence: Synthetic polynucleotide"
caggtgcagctggtgcagtcaggcgccgaagtgaagaaacccggcgctagtgtgaaagtctcttgtaaagctagtggctacaccttcactagctataatatgcactgggttcgccaggccccagggcagggcctcgagtggatcggcgatatctaccccgggaacggcgacactagttataatcagaagtttaagggtagagctactatgaccgccgataagtctactagcaccgtctatatggaactgagttccctgaggtctgaggacaccgccgtctactactgcgctagagtgggcggagccttccctatggactactggggtcaaggcaccctggtcaccgtgtctagcgctagcactaagggcccgtccgtgttccccctggcaccttgtagccggagcactagcgaatccaccgctgccctcggctgcctggtcaaggattacttcccggagcccgtgaccgtgtcctggaacagcggagccctgacctccggagtgcacaccttccccgctgtgctgcagagctccgggctgtactcgctgtcgtcggtggtcacggtgccttcatctagcctgggtaccaagacctacacttgcaacgtggaccacaagccttccaacactaaggtggacaagcgcgtcgaatcgaagtacggcccaccgtgcccgccttgtcccgcgccggagttcctcggcggtccctcggtctttctgttcccaccgaagcccaaggacactttgatgatttcccgcacccctgaagtgacatgcgtggtcgtggacgtgtcacaggaagatccggaggtgcagttcaattggtacgtggatggcgtcgaggtgcacaacgccaaaaccaagccgagggaggagcagttcaactccacttaccgcgtcgtgtccgtgctgacggtgctgcatcaggactggctgaacgggaaggagtacaagtgcaaagtgtccaacaagggacttcctagctcaatcgaaaagaccatctcgaaagccaagggacagccccgggaaccccaagtgtataccctgccaccgagccaggaagaaatgactaagaaccaagtctcattgacttgccttgtgaagggcttctacccatcggatatcgccgtggaatgggagtccaacggccagccggaaaacaactacaagaccacccctccggtgctggactcagacggatccttcttcctctactcgcggctgaccgtggataagagcagatggcaggagggaaatgtgttcagctgttctgtgatgcatgaagccctgcacaaccactacactcagaagtccctgtccctctccctggga

SEQ ID NO: 20 - protein, 111 aa, Artificial Sequence
  source: /note="Description of Artificial Sequence: Synthetic polypeptide"
DIVLTQSPDSLAVSLGERATINCRASESVEYYGTSLMQWYQQKPGQPPKLLIYAASNVESGVPDRFSGSGSGTDFTLTISSLQAEDVAVYYCQQSRKDPSTFGGGTKVEIK

SEQ ID NO: 21 - DNA, 333 bp, Artificial Sequence
  source: /note="Description of Artificial Sequence: Synthetic polynucleotide"
gatatcgtcctgactcagtcacccgatagcctggccgtcagcctgggcgagcgggctactattaactgtagagctagtgaatcagtcgagtactacggcactagcctgatgcagtggtatcagcagaagcccggtcaaccccctaagctgctgatctacgccgcctctaacgtggaatcaggcgtgcccgataggtttagcggtagcggtagtggcaccgacttcaccctgactattagtagcctgcaggccgaggacgtggccgtctactactgtcagcagtctaggaaggaccctagcaccttcggcggaggcactaaggtcgagattaag

SEQ ID NO: 22 - protein, 218 aa, Artificial Sequence
  source: /note="Description of Artificial Sequence: Synthetic polypeptide"
DIVLTQSPDSLAVSLGERATINCRASESVEYYGTSLMQWYQQKPGQPPKLLIYAASNVESGVPDRFSGSGSGTDFTLTISSLQAEDVAVYYCQQSRKDPSTFGGGTKVEIKRTVAAPSVFIFPPSDEQLKSGTASVVCLLNNFYPREAKVQWKVDNALQSGNSQESVTEQDSKDSTYSLSSTLTLSKADYEKHKVYACEVTHQGLSSPVTKSFNRGEC

SEQ ID NO: 23 - DNA, 654 bp, Artificial Sequence
  source: /note="Description of Artificial Sequence: Synthetic polynucleotide"
gatatcgtcctgactcagtcacccgatagcctggccgtcagcctgggcgagcgggctactattaactgtagagctagtgaatcagtcgagtactacggcactagcctgatgcagtggtatcagcagaagcccggtcaaccccctaagctgctgatctacgccgcctctaacgtggaatcaggcgtgcccgataggtttagcggtagcggtagtggcaccgacttcaccctgactattagtagcctgcaggccgaggacgtggccgtctactactgtcagcagtctaggaaggaccctagcaccttcggcggaggcactaaggtcgagattaagcgtacggtggccgctcccagcgtgttcatcttcccccccagcgacgagcagctgaagagcggcaccgccagcgtggtgtgcctgctgaacaacttctacccccgggaggccaaggtgcagtggaaggtggacaacgccctgcagagcggcaacagccaggagagcgtcaccgagcaggacagcaaggactccacctacagcctgagcagcaccctgaccctgagcaaggccgactacgagaagcataaggtgtacgcctgcgaggtgacccaccagggcctgtccagccccgtgaccaagagcttcaacaggggcgagtgc

SEQ ID NO: 24 - protein, 17 aa, Artificial Sequence
  source: /note="Description of Artificial Sequence: Synthetic peptide"
DIYPGSGDTSYNQKFKG

SEQ ID NO: 25 - protein, 6 aa, Artificial Sequence
  source: /note="Description of Artificial Sequence: Synthetic peptide"
YPGSGD

SEQ ID NO: 26 - protein, 118 aa, Artificial Sequence
  source: /note="Description of Artificial Sequence: Synthetic polypeptide"
QVQLVQSGAEVKKPGASVKVSCKASGYTFTSYNMHWVRQAPGQGLEWIGDIYPGSGDTSYNQKFKGRATMTADKSTSTVYMELSSLRSEDTAVYYCARVGGAFPMDYWGQGTLVTVSS

SEQ ID NO: 27 - DNA, 354 bp, Artificial Sequence
  source: /note="Description of Artificial Sequence: Synthetic polynucleotide"
caggtgcagctggtgcagtcaggcgccgaagtgaagaaacccggcgctagtgtgaaagttagctgtaaagctagtggctacaccttcactagctataatatgcactgggttcgccaggccccaggtcaaggcctcgagtggatcggcgatatctaccccggtagcggcgacactagttataatcagaagtttaagggtagagctactatgaccgccgataagtctactagcaccgtctatatggaactgagttccctgaggtctgaagataccgccgtctactactgcgctagagtgggcggagccttccctatggactactggggtcaaggcaccctggtcaccgtgtctagc

SEQ ID NO: 28 - protein, 444 aa, Artificial Sequence
  source: /note="Description of Artificial Sequence: Synthetic polypeptide"
QVQLVQSGAEVKKPGASVKVSCKASGYTFTSYNMHWVRQAPGQGLEWIGDIYPGSGDTSYNQKFKGRATMTADKSTSTVYMELSSLRSEDTAVYYCARVGGAFPMDYWGQGTLVTVSSASTKGPSVFPLAPCSRSTSESTAALGCLVKDYFPEPVTVSWNSGALTSGVHTFPAVLQSSGLYSLSSVVTVPSSSLGTKTYTCNVDHKPSNTKVDKRVESKYGPPCPPCPAPEFLGGPSVFLFPPKPKDTLMISRTPEVTCVVVDVSQEDPEVQFNWYVDGVEVHNAKTKPREEQFNSTYRVVSVLTVLHQDWLNGKEYKCKVSNKGLPSSIEKTISKAKGQPREPQVYTLPPSQEEMTKNQVSLTCLVKGFYPSDIAVEWESNGQPENNYKTTPPVLDSDGSFFLYSRLTVDKSRWQEGNVFSCSVMHEALHNHYTQKSLSLSLG

SEQ ID NO: 29 - DNA, 1332 bp, Artificial Sequence
  source: /note="Description of Artificial Sequence: Synthetic polynucleotide"
caggtgcagctggtgcagtcaggcgccgaagtgaagaaacccggcgctagtgtgaaagttagctgtaaagctagtggctacaccttcactagctataatatgcactgggttcgccaggccccaggtcaaggcctcgagtggatcggcgatatctaccccggtagcggcgacactagttataatcagaagtttaagggtagagctactatgaccgccgataagtctactagcaccgtctatatggaactgagttccctgaggtctgaagataccgccgtctactactgcgctagagtgggcggagccttccctatggactactggggtcaaggcaccctggtcaccgtgtctagcgctagcactaagggcccgtccgtgttccccctggcaccttgtagccggagcactagcgaatccaccgctgccctcggctgcctggtcaaggattacttcccggagcccgtgaccgtgtcctggaacagcggagccctgacctccggagtgcacaccttccccgctgtgctgcagagctccgggctgtactcgctgtcgtcggtggtcacggtgccttcatctagcctgggtaccaagacctacacttgcaacgtggaccacaagccttccaacactaaggtggacaagcgcgtcgaatcgaagtacggcccaccgtgcccgccttgtcccgcgccggagttcctcggcggtccctcggtctttctgttcccaccgaagcccaaggacactttgatgatttcccgcacccctgaagtgacatgcgtggtcgtggacgtgtcacaggaagatccggaggtgcagttcaattggtacgtggatggcgtcgaggtgcacaacgccaaaaccaagccgagggaggagcagttcaactccacttaccgcgtcgtgtccgtgctgacggtgctgcatcaggactggctgaacgggaaggagtacaagtgcaaagtgtccaacaagggacttcctagctcaatcgaaaagaccatctcgaaagccaagggacagccccgggaaccccaagtgtataccctgccaccgagccaggaagaaatgactaagaaccaagtctcattgacttgccttgtgaagggcttctacccatcggatatcgccgtggaatgggagtccaacggccagccggaaaacaactacaagaccacccctccggtgctggactcagacggatccttcttcctctactcgcggctgaccgtggataagagcagatggcaggagggaaatgtgttcagctgttctgtgatgcatgaagccctgcacaaccactacactcagaagtccctgtccctctccctggga

SEQ ID NO: 30 - protein, 17 aa, Artificial Sequence
  source: /note="Description of Artificial Sequence: Synthetic peptide"
DIYPGQGDTSYNQKFKG

SEQ ID NO: 31 - protein, 6 aa, Artificial Sequence
  source: /note="Description of Artificial Sequence: Synthetic peptide"
YPGQGD

SEQ ID NO: 32 - protein, 118 aa, Artificial Sequence
  source: /note="Description of Artificial Sequence: Synthetic polypeptide"
QVQLVQSGAEVKKPGASVKVSCKASGYTFTSYNMHWVRQAPGQGLEWIGDIYPGQGDTSYNQKFKGRATMTADKSTSTVYMELSSLRSEDTAVYYCARVGGAFPMDYWGQGTLVTVSS

SEQ ID NO: 33 - DNA, 354 bp, Artificial Sequence
  source: /note="Description of Artificial Sequence: Synthetic polynucleotide"
caggtgcagctggtgcagtcaggcgccgaagtgaagaaacccggcgctagtgtgaaagttagctgtaaagctagtggctatactttcacttcttataatatgcactgggtccgccaggccccaggtcaaggcctcgagtggatcggcgatatctaccccggtcaaggcgacacttcctataatcagaagtttaagggtagagctactatgaccgccgataagtctacttctaccgtctatatggaactgagttccctgaggtctgaggacaccgccgtctactactgcgctagagtgggcggagccttcccaatggactactggggtcaaggcaccctggtcaccgtgtctagc

SEQ ID NO: 34 - protein, 444 aa, Artificial Sequence
  source: /note="Description of Artificial Sequence: Synthetic polypeptide"
QVQLVQSGAEVKKPGASVKVSCKASGYTFTSYNMHWVRQAPGQGLEWIGDIYPGQGDTSYNQKFKGRATMTADKSTSTVYMELSSLRSEDTAVYYCARVGGAFPMDYWGQGTLVTVSSASTKGPSVFPLAPCSRSTSESTAALGCLVKDYFPEPVTVSWNSGALTSGVHTFPAVLQSSGLYSLSSVVTVPSSSLGTKTYTCNVDHKPSNTKVDKRVESKYGPPCPPCPAPEFLGGPSVFLFPPKPKDTLMISRTPEVTCVVVDVSQEDPEVQFNWYVDGVEVHNAKTKPREEQFNSTYRVVSVLTVLHQDWLNGKEYKCKVSNKGLPSSIEKTISKAKGQPREPQVYTLPPSQEEMTKNQVSLTCLVKGFYPSDIAVEWESNGQPENNYKTTPPVLDSDGSFFLYSRLTVDKSRWQEGNVFSCSVMHEALHNHYTQKSLSLSLG

SEQ ID NO: 35 - DNA, 1332 bp, Artificial Sequence
  source: /note="Description of Artificial Sequence: Synthetic polynucleotide"
caggtgcagctggtgcagtcaggcgccgaagtgaagaaacccggcgctagtgtgaaagttagctgtaaagctagtggctatactttcacttcttataatatgcactgggtccgccaggccccaggtcaaggcctcgagtggatcggcgatatctaccccggtcaaggcgacacttcctataatcagaagtttaagggtagagctactatgaccgccgataagtctacttctaccgtctatatggaactgagttccctgaggtctgaggacaccgccgtctactactgcgctagagtgggcggagccttcccaatggactactggggtcaaggcaccctggtcaccgtgtctagcgctagcactaagggcccgtccgtgttccccctggcaccttgtagccggagcactagcgaatccaccgctgccctcggctgcctggtcaaggattacttcccggagcccgtgaccgtgtcctggaacagcggagccctgacctccggagtgcacaccttccccgctgtgctgcagagctccgggctgtactcgctgtcgtcggtggtcacggtgccttcatctagcctgggtaccaagacctacacttgcaacgtggaccacaagccttccaacactaaggtggacaagcgcgtcgaatcgaagtacggcccaccgtgcccgccttgtcccgcgccggagttcctcggcggtccctcggtctttctgttcccaccgaagcccaaggacactttgatgatttcccgcacccctgaagtgacatgcgtggtcgtggacgtgtcacaggaagatccggaggtgcagttcaattggtacgtggatggcgtcgaggtgcacaacgccaaaaccaagccgagggaggagcagttcaactccacttaccgcgtcgtgtccgtgctgacggtgctgcatcaggactggctgaacgggaaggagtacaagtgcaaagtgtccaacaagggacttcctagctcaatcgaaaagaccatctcgaaagccaagggacagccccgggaaccccaagtgtataccctgccaccgagccaggaagaaatgactaagaaccaagtctcattgacttgccttgtgaagggcttctacccatcggatatcgccgtggaatgggagtccaacggccagccggaaaacaactacaagaccacccctccggtgctggactcagacggatccttcttcctctactcgcggctgaccgtggataagagcagatggcaggagggaaatgtgttcagctgttctgtgatgcatgaagccctgcacaaccactacactcagaagtccctgtccctctccctggga

SEQ ID NO: 36 - protein, 118 aa, Artificial Sequence
  source: /note="Description of Artificial Sequence: Synthetic polypeptide"
QVQLVQSGAEVKKPGASVKVSCKASGYTFTSYNMHWIRQAPGQGLEWIGDIYPGNGDTSYNQKFKGRATLTADKSTSTVYMELSSLRSEDTAVYYCARVGGAFPMDYWGQGTLVTVSS

SEQ ID NO: 37 - DNA, 354 bp, Artificial Sequence
  source: /note="Description of Artificial Sequence: Synthetic polynucleotide"
caggtgcagctggtgcagtcaggcgccgaagtgaagaaacccggcgctagtgtgaaagtttcttgtaaagctagtggctacaccttcactagctataatatgcactggattagacaggccccagggcagggcctcgagtggatcggcgatatctaccccgggaacggcgacactagttataatcagaagtttaagggtagagctaccctgaccgccgataagtctactagcaccgtctatatggaactgagttccctgaggtctgaggacaccgccgtctactactgcgctagagtgggcggagccttccctatggactactgggggcagggcaccctggtcaccgtgtctagc

SEQ ID NO: 38 - protein, 444 aa, Artificial Sequence
  source: /note="Description of Artificial Sequence: Synthetic polypeptide"
QVQLVQSGAEVKKPGASVKVSCKASGYTFTSYNMHWIRQAPGQGLEWIGDIYPGNGDTSYNQKFKGRATLTADKSTSTVYMELSSLRSEDTAVYYCARVGGAFPMDYWGQGTLVTVSSASTKGPSVFPLAPCSRSTSESTAALGCLVKDYFPEPVTVSWNSGALTSGVHTFPAVLQSSGLYSLSSVVTVPSSSLGTKTYTCNVDHKPSNTKVDKRVESKYGPPCPPCPAPEFLGGPSVFLFPPKPKDTLMISRTPEVTCVVVDVSQEDPEVQFNWYVDGVEVHNAKTKPREEQFNSTYRVVSVLTVLHQDWLNGKEYKCKVSNKGLPSSIEKTISKAKGQPREPQVYTLPPSQEEMTKNQVSLTCLVKGFYPSDIAVEWESNGQPENNYKTTPPVLDSDGSFFLYSRLTVDKSRWQEGNVFSCSVMHEALHNHYTQKSLSLSLG

SEQ ID NO: 39 - DNA, 1332 bp, Artificial Sequence
  source: /note="Description of Artificial Sequence: Synthetic polynucleotide"
caggtgcagctggtgcagtcaggcgccgaagtgaagaaacccggcgctagtgtgaaagtttcttgtaaagctagtggctacaccttcactagctataatatgcactggattagacaggccccagggcagggcctcgagtggatcggcgatatctaccccgggaacggcgacactagttataatcagaagtttaagggtagagctaccctgaccgccgataagtctactagcaccgtctatatggaactgagttccctgaggtctgaggacaccgccgtctactactgcgctagagtgggcggagccttccctatggactactgggggcagggcaccctggtcaccgtgtctagcgctagcactaagggcccgtccgtgttccccctggcaccttgtagccggagcactagcgaatccaccgctgccctcggctgcctggtcaaggattacttcccggagcccgtgaccgtgtcctggaacagcggagccctgacctccggagtgcacaccttccccgctgtgctgcagagctccgggctgtactcgctgtcgtcggtggtcacggtgccttcatctagcctgggtaccaagacctacacttgcaacgtggaccacaagccttccaacactaaggtggacaagcgcgtcgaatcgaagtacggcccaccgtgcccgccttgtcccgcgccggagttcctcggcggtccctcggtctttctgttcccaccgaagcccaaggacactttgatgatttcccgcacccctgaagtgacatgcgtggtcgtggacgtgtcacaggaagatccggaggtgcagttcaattggtacgtggatggcgtcgaggtgcacaacgccaaaaccaagccgagggaggagcagttcaactccacttaccgcgtcgtgtccgtgctgacggtgctgcatcaggactggctgaacgggaaggagtacaagtgcaaagtgtccaacaagggacttcctagctcaatcgaaaagaccatctcgaaagccaagggacagccccgggaaccccaagtgtataccctgccaccgagccaggaagaaatgactaagaaccaagtctcattgacttgccttgtgaagggcttctacccatcggatatcgccgtggaatgggagtccaacggccagccggaaaacaactacaagaccacccctccggtgctggactcagacggatccttcttcctctactcgcggctgaccgtggataagagcagatggcaggagggaaatgtgttcagctgttctgtgatgcatgaagccctgcacaaccactacactcagaagtccctgtccctctccctggga

SEQ ID NO: 40 - protein, 111 aa, Artificial Sequence
  source: /note="Description of Artificial Sequence: Synthetic polypeptide"
DIVLTQSPDSLAVSLGERATINCRASESVEYYGTSLMQWYQQKPGQPPKLLIYAASNVESGVPDRFSGSGSGTDFTLTISSLQAEDVAVYFCQQSRKDPSTFGGGTKVEIK

SEQ ID NO: 41 - DNA, 333 bp, Artificial Sequence
  source: /note="Description of Artificial Sequence: Synthetic polynucleotide"
gatatcgtcctgactcagtcacccgatagcctggccgtcagcctgggcgagcgggctactattaactgtagagctagtgaatcagtcgagtactacggcactagcctgatgcagtggtatcagcagaagcccggtcaaccccctaagctgctgatctacgccgcctctaacgtggaatcaggcgtgcccgataggtttagcggtagcggtagtggcaccgacttcaccctgactattagtagcctgcaggccgaggacgtggccgtctacttctgtcagcagtctaggaaggaccctagcaccttcggcggaggcactaaggtcgagattaag

SEQ ID NO: 42 - protein, 218 aa, Artificial Sequence
  source: /note="Description of Artificial Sequence: Synthetic polypeptide"
DIVLTQSPDSLAVSLGERATINCRASESVEYYGTSLMQWYQQKPGQPPKLLIYAASNVESGVPDRFSGSGSGTDFTLTISSLQAEDVAVYFCQQSRKDPSTFGGGTKVEIKRTVAAPSVFIFPPSDEQLKSGTASVVCLLNNFYPREAKVQWKVDNALQSGNSQESVTEQDSKDSTYSLSSTLTLSKADYEKHKVYACEVTHQGLSSPVTKSFNRGEC

SEQ ID NO: 43 - DNA, 654 bp, Artificial Sequence
  source: /note="Description of Artificial Sequence: Synthetic polynucleotide"
gatatcgtcctgactcagtcacccgatagcctggccgtcagcctgggcgagcgggctactattaactgtagagctagtgaatcagtcgagtactacggcactagcctgatgcagtggtatcagcagaagcccggtcaaccccctaagctgctgatctacgccgcctctaacgtggaatcaggcgtgcccgataggtttagcggtagcggtagtggcaccgacttcaccctgactattagtagcctgcaggccgaggacgtggccgtctacttctgtcagcagtctaggaaggaccctagcaccttcggcggaggcactaaggtcgagattaagcgtacggtggccgctcccagcgtgttcatcttcccccccagcgacgagcagctgaagagcggcaccgccagcgtggtgtgcctgctgaacaacttctacccccgggaggccaaggtgcagtggaaggtggacaacgccctgcagagcggcaacagccaggagagcgtcaccgagcaggacagcaaggactccacctacagcctgagcagcaccctgaccctgagcaaggccgactacgagaagcataaggtgtacgcctgcgaggtgacccaccagggcctgtccagccccgtgaccaagagcttcaacaggggcgagtgc

SEQ ID NO: 44 - protein, 118 aa, Artificial Sequence
  source: /note="Description of Artificial Sequence: Synthetic polypeptide"
QVQLVQSGAEVKKPGASVKVSCKASGYTFTSYNMHWIRQAPGQGLEWIGDIYPGSGDTSYNQKFKGRATLTADKSTSTVYMELSSLRSEDTAVYYCARVGGAFPMDYWGQGTLVTVSS

SEQ ID NO: 45 - DNA, 354 bp, Artificial Sequence
  source: /note="Description of Artificial Sequence: Synthetic polynucleotide"
caggtgcagctggtgcagtcaggcgccgaagtgaagaaacccggcgcaagcgttaaagtctcatgtaaagctagtggctacaccttcactagctataatatgcactggattagacaggccccagggcaaggcctggagtggatcggcgatatctaccccggtagcggcgacactagttataatcagaagtttaagggtagagctaccctgaccgccgataagtctactagcaccgtctatatggaactgagttccctgaggagtgaagacaccgccgtctactactgcgctagagtgggcggagccttccctatggactactggggtcaaggcaccctggtcaccgtgtcaagc

SEQ ID NO: 46 - protein, 444 aa, Artificial Sequence
  source: /note="Description of Artificial Sequence: Synthetic polypeptide"
QVQLVQSGAEVKKPGASVKVSCKASGYTFTSYNMHWIRQAPGQGLEWIGDIYPGSGDTSYNQKFKGRATLTADKSTSTVYMELSSLRSEDTAVYYCARVGGAFPMDYWGQGTLVTVSSASTKGPSVFPLAPCSRSTSESTAALGCLVKDYFPEPVTVSWNSGALTSGVHTFPAVLQSSGLYSLSSVVTVPSSSLGTKTYTCNVDHKPSNTKVDKRVESKYGPPCPPCPAPEFLGGPSVFLFPPKPKDTLMISRTPEVTCVVVDVSQEDPEVQFNWYVDGVEVHNAKTKPREEQFNSTYRVVSVLTVLHQDWLNGKEYKCKVSNKGLPSSIEKTISKAKGQPREPQVYTLPPSQEEMTKNQVSLTCLVKGFYPSDIAVEWESNGQPENNYKTTPPVLDSDGSFFLYSRLTVDKSRWQEGNVFSCSVMHEALHNHYTQKSLSLSLG

SEQ ID NO: 47 - DNA, 1332 bp, Artificial Sequence
  source: /note="Description of Artificial Sequence: Synthetic polynucleotide"
caggtgcagctggtgcagtcaggcgccgaagtgaagaaacccggcgcaagcgttaaagtctcatgtaaagctagtggctacaccttcactagctataatatgcactggattagacaggccccagggcaaggcctggagtggatcggcgatatctaccccggtagcggcgacactagttataatcagaagtttaagggtagagctaccctgaccgccgataagtctactagcaccgtctatatggaactgagttccctgaggagtgaagacaccgccgtctactactgcgctagagtgggcggagccttccctatggactactggggtcaaggcaccctggtcaccgtgtcaagcgctagcactaagggcccgtccgtgttccccctggcaccttgtagccggagcactagcgaatccaccgctgccctcggctgcctggtcaaggattacttcccggagcccgtgaccgtgtcctggaacagcggagccctgacctccggagtgcacaccttccccgctgtgctgcagagctccgggctgtactcgctgtcgtcggtggtcacggtgccttcatctagcctgggtaccaagacctacacttgcaacgtggaccacaagccttccaacactaaggtggacaagcgcgtcgaatcgaagtacggcccaccgtgcccgccttgtcccgcgccggagttcctcggcggtccctcggtctttctgttcccaccgaagcccaaggacactttgatgatttcccgcacccctgaagtgacatgcgtggtcgtggacgtgtcacaggaagatccggaggtgcagttcaattggtacgtggatggcgtcgaggtgcacaacgccaaaaccaagccgagggaggagcagttcaactccacttaccgcgtcgtgtccgtgctgacggtgctgcatcaggactggctgaacgggaaggagtacaagtgcaaagtgtccaacaagggacttcctagctcaatcgaaaagaccatctcgaaagccaagggacagccccgggaaccccaagtgtataccctgccaccgagccaggaagaaatgactaagaaccaagtctcattgacttgccttgtgaagggcttctacccatcggatatcgccgtggaatgggagtccaacggccagccggaaaacaactacaagaccacccctccggtgctggactcagacggatccttcttcctctactcgcggctgaccgtggataagagcagatggcaggagggaaatgtgttcagctgttctgtgatgcatgaagccctgcacaaccactacactcagaagtccctgtccctctccctggga

SEQ ID NO: 48 - protein, 118 aa, Artificial Sequence
  source: /note="Description of Artificial Sequence: Synthetic polypeptide"
QVQLVQSGAEVKKPGASVKVSCKASGYTFTSYNMHWIRQAPGQGLEWIGDIYPGQGDTSYNQKFKGRATLTADKSTSTVYMELSSLRSEDTAVYYCARVGGAFPMDYWGQGTLVTVSS

SEQ ID NO: 49 - DNA, 354 bp, Artificial Sequence
  source: /note="Description of Artificial Sequence: Synthetic polynucleotide"
caggtgcagctggtgcagtcaggcgccgaagtgaagaaacccggcgctagtgtgaaagtctcttgtaaagctagtggctacaccttcactagctataatatgcactggattagacaggccccaggtcaaggcctcgagtggatcggcgatatctaccccggtcaaggcgacactagttataatcagaagtttaagggtagagctaccctgaccgccgataagtctactagcaccgtctatatggaactgagttccctgaggtctgaggacaccgccgtctactactgcgctagagtgggcggagccttccctatggactactggggtcaaggcaccctggtcaccgtgtctagc

SEQ ID NO: 50 - protein, 444 aa, Artificial Sequence
  source: /note="Description of Artificial Sequence: Synthetic polypeptide"
QVQLVQSGAEVKKPGASVKVSCKASGYTFTSYNMHWIRQAPGQGLEWIGDIYPGQGDTSYNQKFKGRATLTADKSTSTVYMELSSLRSEDTAVYYCARVGGAFPMDYWGQGTLVTVSSASTKGPSVFPLAPCSRSTSESTAALGCLVKDYFPEPVTVSWNSGALTSGVHTFPAVLQSSGLYSLSSVVTVPSSSLGTKTYTCNVDHKPSNTKVDKRVESKYGPPCPPCPAPEFLGGPSVFLFPPKPKDTLMISRTPEVTCVVVDVSQEDPEVQFNWYVDGVEVHNAKTKPREEQFNSTYRVVSVLTVLHQDWLNGKEYKCKVSNKGLPSSIEKTISKAKGQPREPQVYTLPPSQEEMTKNQVSLTCLVKGFYPSDIAVEWESNGQPENNYKTTPPVLDSDGSFFLYSRLTVDKSRWQEGNVFSCSVMHEALHNHYTQKSLSLSLG

SEQ ID NO: 51 - DNA, 1332 bp, Artificial Sequence
  source: /note="Description of Artificial Sequence: Synthetic polynucleotide"
caggtgcagctggtgcagtcaggcgccgaagtgaagaaacccggcgctagtgtgaaagtctcttgtaaagctagtggctacaccttcactagctataatatgcactggattagacaggccccaggtcaaggcctcgagtggatcggcgatatctaccccggtcaaggcgacactagttataatcagaagtttaagggtagagctaccctgaccgccgataagtctactagcaccgtctatatggaactgagttccctgaggtctgaggacaccgccgtctactactgcgctagagtgggcggagccttccctatggactactggggtcaaggcaccctggtcaccgtgtctagcgctagcactaagggcccgtccgtgttccccctggcaccttgtagccggagcactagcgaatccaccgctgccctcggctgcctggtcaaggattacttcccggagcccgtgaccgtgtcctggaacagcggagccctgacctccggagtgcacaccttccccgctgtgctgcagagctccgggctgtactcgctgtcgtcggtggtcacggtgccttcatctagcctgggtaccaagacctacacttgcaacgtggaccacaagccttccaacactaaggtggacaagcgcgtcgaatcgaagtacggcccaccgtgcccgccttgtcccgcgccggagttcctcggcggtccctcggtctttctgttcccaccgaagcccaaggacactttgatgatttcccgcacccctgaagtgacatgcgtggtcgtggacgtgtcacaggaagatccggaggtgcagttcaattggtacgtggatggcgtcgaggtgcacaacgccaaaaccaagccgagggaggagcagttcaactccacttaccgcgtcgtgtccgtgctgacggtgctgcatcaggactggctgaacgggaaggagtacaagtgcaaagtgtccaacaagggacttcctagctcaatcgaaaagaccatctcgaaagccaagggacagccccgggaaccccaagtgtataccctgccaccgagccaggaagaaatgactaagaaccaagtctcattgacttgccttgtgaagggcttctacccatcggatatcgccgtggaatgggagtccaacggccagccggaaaacaactacaagaccacccctccggtgctggactcagacggatccttcttcctctactcgcggctgaccgtggataagagcagatggcaggagggaaatgtgttcagctgttctgtgatgcatgaagccctgcacaaccactacactcagaagtccctgtccctctccctggga

SEQ ID NO: 52 - protein, 118 aa, Artificial Sequence
  source: /note="Description of Artificial Sequence: Synthetic polypeptide"
QVQLVQSGAEVKKPGSSVKVSCKASGYTFTSYNMHWVRQAPGQGLEWMGDIYPGNGDTSYNQKFKGRVTITADKSTSTVYMELSSLRSEDTAVYYCARVGGAFPMDYWGQGTTVTVSS

SEQ ID NO: 53 - DNA, 354 bp, Artificial Sequence
  source: /note="Description of Artificial Sequence: Synthetic polynucleotide"
caggtgcagctggtgcagtcaggcgccgaagtgaagaaacccggctctagcgtgaaagtttcttgtaaagctagtggctacaccttcactagctataatatgcactgggttcgccaggccccagggcaaggcctcgagtggatgggcgatatctaccccgggaacggcgacactagttataatcagaagtttaagggtagagtcactatcaccgccgataagtctactagcaccgtctatatggaactgagttccctgaggtctgaggacaccgccgtctactactgcgctagagtgggcggagccttccctatggactactggggtcaaggcactaccgtgaccgtgtctagc

SEQ ID NO: 54 - protein, 444 aa, Artificial Sequence
  source: /note="Description of Artificial Sequence: Synthetic polypeptide"
QVQLVQSGAEVKKPGSSVKVSCKASGYTFTSYNMHWVRQAPGQGLEWMGDIYPGNGDTSYNQKFKGRVTITADKSTSTVYMELSSLRSEDTAVYYCARVGGAFPMDYWGQGTTVTVSSASTKGPSVFPLAPCSRSTSESTAALGCLVKDYFPEPVTVSWNSGALTSGVHTFPAVLQSSGLYSLSSVVTVPSSSLGTKTYTCNVDHKPSNTKVDKRVESKYGPPCPPCPAPEFLGGPSVFLFPPKPKDTLMISRTPEVTCVVVDVSQEDPEVQFNWYVDGVEVHNAKTKPREEQFNSTYRVVSVLTVLHQDWLNGKEYKCKVSNKGLPSSIEKTISKAKGQPREPQVYTLPPSQEEMTKNQVSLTCLVKGFYPSDIAVEWESNGQPENNYKTTPPVLDSDGSFFLYSRLTVDKSRWQEGNVFSCSVMHEALHNHYTQKSLSLSLG

SEQ ID NO: 55 - DNA, 1332 bp, Artificial Sequence
  source: /note="Description of Artificial Sequence: Synthetic polynucleotide"
caggtgcagctggtgcagtcaggcgccgaagtgaagaaacccggctctagcgtgaaagtttcttgtaaagctagtggctacaccttcactagctataatatgcactgggttcgccaggccccagggcaaggcctcgagtggatgggcgatatctaccccgggaacggcgacactagttataatcagaagtttaagggtagagtcactatcaccgccgataagtctactagcaccgtctatatggaactgagttccctgaggtctgaggacaccgccgtctactactgcgctagagtgggcggagccttccctatggactactggggtcaaggcactaccgtgaccgtgtctagcgctagcactaagggcccgtccgtgttccccctggcaccttgtagccggagcactagcgaatccaccgctgccctcggctgcctggtcaaggattacttcccggagcccgtgaccgtgtcctggaacagcggagccctgacctccggagtgcacaccttccccgctgtgctgcagagctccgggctgtactcgctgtcgtcggtggtcacggtgccttcatctagcctgggtaccaagacctacacttgcaacgtggaccacaagccttccaacactaaggtggacaagcgcgtcgaatcgaagtacggcccaccgtgcccgccttgtcccgcgccggagttcctcggcggtccctcggtctttctgttcccaccgaagcccaaggacactttgatgatttcccgcacccctgaagtgacatgcgtggtcgtggacgtgtcacaggaagatccggaggtgcagttcaattggtacgtggatggcgtcgaggtgcacaacgccaaaaccaagccgagggaggagcagttcaactccacttaccgcgtcgtgtccgtgctgacggtgctgcatcaggactggctgaacgggaaggagtacaagtgcaaagtgtccaacaagggacttcctagctcaatcgaaaagaccatctcgaaagccaagggacagccccgggaaccccaagtgtataccctgccaccgagccaggaagaaatgactaagaaccaagtctcattgacttgccttgtgaagggcttctacccatcggatatcgccgtggaatgggagtccaacggccagccggaaaacaactacaagaccacccctccggtgctggactcagacggatccttcttcctctactcgcggctgaccgtggataagagcagatggcaggagggaaatgtgttcagctgttctgtgatgcatgaagccctgcacaaccactacactcagaagtccctgtccctctccctggga

SEQ ID NO: 56 - protein, 111 aa, Artificial Sequence
  source: /note="Description of Artificial Sequence: Synthetic polypeptide"
EIVLTQSPATLSLSPGERATLSCRASESVEYYGTSLMQWYQQKPGQAPRLLIYAASNVESGIPARFSGSGSGTDFTLTISSLEPEDIAVYFCQQSRKDPSTFGGGTKVEIK

SEQ ID NO: 57 - DNA, 333 bp, Artificial Sequence
  source: /note="Description of Artificial Sequence: Synthetic polynucleotide"
gagatcgtcctgactcagtcacccgctaccctgagcctgagccctggcgagagagctacactgagctgtagagctagtgaatcagtcgagtactacggcactagcctgatgcagtggtatcagcagaagcccggtcaagcccctagactgctgatctacgccgcctctaacgtggaatcagggatccccgctaggtttagcggtagcggtagtggcaccgacttcaccctgactatctctagcctggaacccgaggatatcgccgtctacttctgtcagcagtctaggaaggaccctagcaccttcggcggaggcactaaggtcgagattaag

SEQ ID NO: 58 - protein, 218 aa, Artificial Sequence
  source: /note="Description of Artificial Sequence: Synthetic polypeptide"
EIVLTQSPATLSLSPGERATLSCRASESVEYYGTSLMQWYQQKPGQAPRLLIYAASNVESGIPARFSGSGSGTDFTLTISSLEPEDIAVYFCQQSRKDPSTFGGGTKVEIKRTVAAPSVFIFPPSDEQLKSGTASVVCLLNNFYPREAKVQWKVDNALQSGNSQESVTEQDSKDSTYSLSSTLTLSKADYEKHKVYACEVTHQGLSSPVTKSFNRGEC

SEQ ID NO: 59 - DNA, 654 bp, Artificial Sequence
  source: /note="Description of Artificial Sequence: Synthetic polynucleotide"
gagatcgtcctgactcagtcacccgctaccctgagcctgagccctggcgagagagctacactgagctgtagagctagtgaatcagtcgagtactacggcactagcctgatgcagtggtatcagcagaagcccggtcaagcccctagactgctgatctacgccgcctctaacgtggaatcagggatccccgctaggtttagcggtagcggtagtggcaccgacttcaccctgactatctctagcctggaacccgaggatatcgccgtctacttctgtcagcagtctaggaaggaccctagcaccttcggcggaggcactaaggtcgagattaagcgtacggtggccgctcccagcgtgttcatcttcccccccagcgacgagcagctgaagagcggcaccgccagcgtggtgtgcctgctgaacaacttctacccccgggaggccaaggtgcagtggaaggtggacaacgccctgcagagcggcaacagccaggagagcgtcaccgagcaggacagcaaggactccacctacagcctgagcagcaccctgaccctgagcaaggccgactacgagaagcataaggtgtacgcctgcgaggtgacccaccagggcctgtccagccccgtgaccaagagcttcaacaggggcgagtgc

SEQ ID NO: 60 - protein, 118 aa, Artificial Sequence
  source: /note="Description of Artificial Sequence: Synthetic polypeptide"
EVQLVQSGAEVKKPGESLKISCKGSGYTFTSYNMHWVRQMPGKGLEWMGDIYPGNGDTSYNQKFKGQVTISADKSISTVYLQWSSLKASDTAMYYCARVGGAFPMDYWGQGTTVTVSS

SEQ ID NO: 61 - DNA, 354 bp, Artificial Sequence
  source: /note="Description of Artificial Sequence: Synthetic polynucleotide"
gaagtgcagctggtgcagtcaggcgccgaagtgaagaagcccggcgagtcactgaagattagctgtaaaggttcaggctacaccttcactagctataatatgcactgggtccgccagatgcccgggaaaggcctcgagtggatgggcgatatctaccccgggaacggcgacactagttataatcagaagtttaaggggcaagtcacaattagcgccgataagtctattagcaccgtctacctgcagtggtctagcctgaaggctagtgacaccgctatgtactactgcgctagagtgggcggagccttccctatggactactggggtcaaggcactaccgtgaccgtgtctagc

SEQ ID NO: 62 - protein, 444 aa, Artificial Sequence
  source: /note="Description of Artificial Sequence: Synthetic polypeptide"
EVQLVQSGAEVKKPGESLKISCKGSGYTFTSYNMHWVRQMPGKGLEWMGDIYPGNGDTSYNQKFKGQVTISADKSISTVYLQWSSLKASDTAMYYCARVGGAFPMDYWGQGTTVTVSSASTKGPSVFPLAPCSRSTSESTAALGCLVKDYFPEPVTVSWNSGALTSGVHTFPAVLQSSGLYSLSSVVTVPSSSLGTKTYTCNVDHKPSNTKVDKRVESKYGPPCPPCPAPEFLGGPSVFLFPPKPKDTLMISRTPEVTCVVVDVSQEDPEVQFNWYVDGVEVHNAKTKPREEQFNSTYRVVSVLTVLHQDWLNGKEYKCKVSNKGLPSSIEKTISKAKGQPREPQVYTLPPSQEEMTKNQVSLTCLVKGFYPSDIAVEWESNGQPENNYKTTPPVLDSDGSFFLYSRLTVDKSRWQEGNVFSCSVMHEALHNHYTQKSLSLSLG

SEQ ID NO: 63 - DNA, 1332 bp, Artificial Sequence
  source: /note="Description of Artificial Sequence: Synthetic polynucleotide"
gaagtgcagctggtgcagtcaggcgccgaagtgaagaagcccggcgagtcactgaagattagctgtaaaggttcaggctacaccttcactagctataatatgcactgggtccgccagatgcccgggaaaggcctcgagtggatgggcgatatctaccccgggaacggcgacactagttataatcagaagtttaaggggcaagtcacaattagcgccgataagtctattagcaccgtctacctgcagtggtctagcctgaaggctagtgacaccgctatgtactactgcgctagagtgggcggagccttccctatggactactggggtcaaggcactaccgtgaccgtgtctagcgctagcactaagggcccgtccgtgttccccctggcaccttgtagccggagcactagcgaatccaccgctgccctcggctgcctggtcaaggattacttcccggagcccgtgaccgtgtcctggaacagcggagccctgacctccggagtgcacaccttccccgctgtgctgcagagctccgggctgtactcgctgtcgtcggtggtcacggtgccttcatctagcctgggtaccaagacctacacttgcaacgtggaccacaagccttccaacactaaggtggacaagcgcgtcgaatcgaagtacggcccaccgtgcccgccttgtcccgcgccggagttcctcggcggtccctcggtctttctgttcccaccgaagcccaaggacactttgatgatttcccgcacccctgaagtgacatgcgtggtcgtggacgtgtcacaggaagatccggaggtgcagttcaattggtacgtggatggcgtcgaggtgcacaacgccaaaaccaagccgagggaggagcagttcaactccacttaccgcgtcgtgtccgtgctgacggtgctgcatcaggactggctgaacgggaaggagtacaagtgcaaagtgtccaacaagggacttcctagctcaatcgaaaagaccatctcgaaagccaagggacagccccgggaaccccaagtgtataccctgccaccgagccaggaagaaatgactaagaaccaagtctcattgacttgccttgtgaagggcttctacccatcggatatcgccgtggaatgggagtccaacggccagccggaaaacaactacaagaccacccctccggtgctggactcagacggatccttcttcctctactcgcggctgaccgtggataagagcagatggcaggagggaaatgtgttcagctgttctgtgatgcatgaagccctgcacaaccactacactcagaagtccctgtccctctccctggga

SEQ ID NO: 64 - protein, 111 aa, Artificial Sequence
  source: /note="Description of Artificial Sequence: Synthetic polypeptide"
AIQLTQSPSSLSASVGDRVTITCRASESVEYYGTSLMQWYQQKPGKAPKLLIYAASNVESGVPSRFSGSGSGTDFTLTISSLQPEDFATYFCQQSRKDPSTFGGGTKVEIK

SEQ ID NO: 65 - DNA, 333 bp, Artificial Sequence
  source: /note="Description of Artificial Sequence: Synthetic polynucleotide"
gctattcagctgactcagtcacctagtagcctgagcgctagtgtgggcgatagagtgactatcacctgtagagctagtgaatcagtcgagtactacggcactagcctgatgcagtggtatcagcagaagcccgggaaagcccctaagctgctgatctacgccgcctctaacgtggaatcaggcgtgccctctaggtttagcggtagcggtagtggcaccgacttcaccctgactatctctagcctgcagcccgaggacttcgctacctacttctgtcagcagtctaggaaggaccctagcaccttcggcggaggcactaaggtcgagattaag

SEQ ID NO: 66 - protein, 218 aa, Artificial Sequence
  source: /note="Description of Artificial Sequence: Synthetic polypeptide"
AIQLTQSPSSLSASVGDRVTITCRASESVEYYGTSLMQWYQQKPGKAPKLLIYAASNVESGVPSRFSGSGSGTDFTLTISSLQPEDFATYFCQQSRKDPSTFGGGTKVEIKRTVAAPSVFIFPPSDEQLKSGTASVVCLLNNFYPREAKVQWKVDNALQSGNSQESVTEQDSKDSTYSLSSTLTLSKADYEKHKVYACEVTHQGLSSPVTKSFNRGEC

SEQ ID NO: 67 - DNA, 654 bp, Artificial Sequence
  source: /note="Description of Artificial Sequence: Synthetic polynucleotide"
gctattcagctgactcagtcacctagtagcctgagcgctagtgtgggcgatagagtgactatcacctgtagagctagtgaatcagtcgagtactacggcactagcctgatgcagtggtatcagcagaagcccgggaaagcccctaagctgctgatctacgccgcctctaacgtggaatcaggcgtgccctctaggtttagcggtagcggtagtggcaccgacttcaccctgactatctctagcctgcagcccgaggacttcgctacctacttctgtcagcagtctaggaaggaccctagcaccttcggcggaggcactaaggtcgagattaagcgtacggtggccgctcccagcgtgttcatcttcccccccagcgacgagcagctgaagagcggcaccgccagcgtggtgtgcctgctgaacaacttctacccccgggaggccaaggtgcagtggaaggtggacaacgccctgcagagcggcaacagccaggagagcgtcaccgagcaggacagcaaggactccacctacagcctgagcagcaccctgaccctgagcaaggccgactacgagaagcataaggtgtacgcctgcgaggtgacccaccagggcctgtccagccccgtgaccaagagcttcaacaggggcgagtgc

SEQ ID NO: 68 - protein, 118 aa, Artificial Sequence
  source: /note="Description of Artificial Sequence: Synthetic polypeptide"
QVQLVQSGAEVKKPGSSVKVSCKASGYTFTSYNMHWVRQAPGQGLEWMGDIYPGSGDTSYNQKFKGRVTITADKSTSTVYMELSSLRSEDTAVYYCARVGGAFPMDYWGQGTTVTVSS

SEQ ID NO: 69 - DNA, 354 bp, Artificial Sequence
  source: /note="Description of Artificial Sequence: Synthetic polynucleotide"
caggtgcaattggttcagtcaggagcagaagttaagaagccaggatcatccgtcaaggtgtcctgcaaagcatctggctacaccttcaccagctacaatatgcactgggtccgacaagcccctgggcagggcttggagtggatgggagacatttaccccggcagtggtgacacttcctataaccagaagttcaagggccgagtcactattaccgctgacaagtccacctccacagtctacatggaactctcttctctgagatccgaggacactgccgtctattactgcgctcgcgtgggcggtgctttcccaatggactattggggacagggcacaaccgtgaccgtcagctca

SEQ ID NO: 70 - protein, 445 aa, Artificial Sequence
  source: /note="Description of Artificial Sequence: Synthetic polypeptide"
QVQLVQSGAEVKKPGSSVKVSCKASGYTFTSYNMHWVRQAPGQGLEWMGDIYPGSGDTSYNQKFKGRVTITADKSTSTVYMELSSLRSEDTAVYYCARVGGAFPMDYWGQGTTVTVSSASTKGPSVFPLAPCSRSTSESTAALGCLVKDYFPEPVTVSWNSGALTSGVHTFPAVLQSSGLYSLSSVVTVPSSSLGTKTYTCNVDHKPSNTKVDKRVESKYGPPCPPCPAPEFLGGPSVFLFPPKPKDTLMISRTPEVTCVVVDVSQEDPEVQFNWYVDGVEVHNAKTKPREEQFNSTYRVVSVLTVLHQDWLNGKEYKCKVSNKGLPSSIEKTISKAKGQPREPQVYTLPPSQEEMTKNQVSLTCLVKGFYPSDIAVEWESNGQPENNYKTTPPVLDSDGSFFLYSRLTVDKSRWQEGNVFSCSVMHEALHNHYTQKSLSLSLGK

SEQ ID NO: 71 - DNA, 1335 bp, Artificial Sequence
  source: /note="Description of Artificial Sequence: Synthetic polynucleotide"
caggtgcaattggttcagtcaggagcagaagttaagaagccaggatcatccgtcaaggtgtcctgcaaagcatctggctacaccttcaccagctacaatatgcactgggtccgacaagcccctgggcagggcttggagtggatgggagacatttaccccggcagtggtgacacttcctataaccagaagttcaagggccgagtcactattaccgctgacaagtccacctccacagtctacatggaactctcttctctgagatccgaggacactgccgtctattactgcgctcgcgtgggcggtgctttcccaatggactattggggacagggcacaaccgtgaccgtcagctcagcctctacaaagggcccctccgtctttccactcgcgccgtgctctcgctccacctcagagtcaactgccgctctgggttgcctggtcaaggactacttcccagagccggtgacagtgagctggaacagtggggccctgacatccggcgttcataccttccccgcagtcctccagtcctcaggcctgtattccctgagcagcgttgtcacagtgccctccagctctcttggcacgaaaacctacacatgcaacgttgatcataagccgtctaataccaaggtggataaaagagtggagagcaagtacggcccaccctgcccgccttgcccagctccggagttcctgggcggaccatccgttttcttgtttccacccaaacctaaagacactctgatgatttcccgaacccctgaagtgacttgcgttgtggtggacgtctcccaggaggacccagaagtgcaattcaactggtacgtggacggggtggaggtgcacaatgcaaaaaccaaaccaagggaggaacagtttaattcaacatatagggttgtgtctgtgctgacggttctgcatcaggactggctgaacggaaaggaatacaagtgcaaggtgtccaacaaaggactgccaagctctatcgagaaaacaatctctaaggccaagggacaacctagagagccccaagtttacaccctgccaccatcacaggaagagatgaccaaaaatcaggtgagcttgacatgcctggtgaagggcttctaccctagcgatattgcggttgagtgggagtcaaatggccagcctgagaacaactataagactactcctcccgtgctggactccgacgggagctttttcctgtattccaggcttacagtcgataagagcagatggcaagaggggaatgtgttttcctgctccgtgatgcacgaggctctccataaccattatactcagaaaagtctctctctgtcactgggcaaa

SEQ ID NO: 72 - protein, 118 aa, Artificial Sequence
  source: /note="Description of Artificial Sequence: Synthetic polypeptide"
QVQLVQSGAEVKKPGSSVKVSCKASGYTFTSYNMHWVRQAPGQGLEWMGDIYPGQGDTSYNQKFKGRVTITADKSTSTVYMELSSLRSEDTAVYYCARVGGAFPMDYWGQGTTVTVSS

SEQ ID NO: 73 - DNA, 354 bp, Artificial Sequence
  source: /note="Description of Artificial Sequence: Synthetic polynucleotide"
caggtgcaattggttcagtcaggagcagaagttaagaagccaggatcatccgtcaaggtgtcctgcaaagcatctggctacaccttcaccagctacaatatgcactgggtccgacaagcccctgggcagggcttggagtggatgggagacatttaccccggccagggtgacacttcctataaccagaagttcaagggccgagtcactattaccgctgacaagtccacctccacagtctacatggaactctcttctctgagatccgaggacactgccgtctattactgcgctcgcgtgggcggtgctttcccaatggactattggggacagggcacaaccgtgaccgtcagctca

SEQ ID NO: 74 - protein, 445 aa, Artificial Sequence
  source: /note="Description of Artificial Sequence: Synthetic polypeptide"
QVQLVQSGAEVKKPGSSVKVSCKASGYTFTSYNMHWVRQAPGQGLEWMGDIYPGQGDTSYNQKFKGRVTITADKSTSTVYMELSSLRSEDTAVYYCARVGGAFPMDYWGQGTTVTVSSASTKGPSVFPLAPCSRSTSESTAALGCLVKDYFPEPVTVSWNSGALTSGVHTFPAVLQSSGLYSLSSVVTVPSSSLGTKTYTCNVDHKPSNTKVDKRVESKYGPPCPPCPAPEFLGGPSVFLFPPKPKDTLMISRTPEVTCVVVDVSQEDPEVQFNWYVDGVEVHNAKTKPREEQFNSTYRVVSVLTVLHQDWLNGKEYKCKVSNKGLPSSIEKTISKAKGQPREPQVYTLPPSQEEMTKNQVSLTCLVKGFYPSDIAVEWESNGQPENNYKTTPPVLDSDGSFFLYSRLTVDKSRWQEGNVFSCSVMHEALHNHYTQKSLSLSLGK

SEQ ID NO: 75 - DNA, 1335 bp, Artificial Sequence
  source: /note="Description of Artificial Sequence: Synthetic polynucleotide"
caggtgcaattggttcagtcaggagcagaagttaagaagccaggatcatccgtcaaggtgtcctgcaaagcatctggctacaccttcaccagctacaatatgcactgggtccgacaagcccctgggcagggcttggagtggatgggagacatttaccccggccagggtgacacttcctataaccagaagttcaagggccgagtcactattaccgctgacaagtccacctccacagtctacatggaactctcttctctgagatccgaggacactgccgtctattactgcgctcgcgtgggcggtgctttcccaatggactattggggacagggcacaaccgtgaccgtcagctcagcctctacaaagggcccctccgtctttccactcgcgccgtgctctcgctccacctcagagtcaactgccgctctgggttgcctggtcaaggactacttcccagagccggtgacagtgagctggaacagtggggccctgacatccggcgttcataccttccccgcagtcctccagtcctcaggcctgtattccctgagcagcgttgtcacagtgccctccagctctcttggcacgaaaacctacacatgcaacgttgatcataagccgtctaataccaaggtggataaaagagtggagagcaagtacggcccaccctgcccgccttgcccagctccggagttcctgggcggaccatccgttttcttgtttccacccaaacctaaagacactctgatgatttcccgaacccctgaagtgacttgcgttgtggtggacgtctcccaggaggacccagaagtgcaattcaactggtacgtggacggggtggaggtgcacaatgcaaaaaccaaaccaagggaggaacagtttaattcaacatatagggttgtgtctgtgctgacggttctgcatcaggactggctgaacggaaaggaatacaagtgcaaggtgtccaacaaaggactgccaagctctatcgagaaaacaatctctaaggccaagggacaacctagagagccccaagtttacaccctgccaccatcacaggaagagatgaccaaaaatcaggtgagcttgacatgcctggtgaagggcttctaccctagcgatattgcggttgagtgggagtcaaatggccagcctgagaacaactataagactactcctcccgtgctggactccgacgggagctttttcctgtattccaggcttacagtcgataagagcagatggcaagaggggaatgtgttttcctgctccgtgatgcacgaggctctccataaccattatactcagaaaagtctctctctgtcactgggcaaa

SEQ ID NO: 76 - protein, 118 aa, Artificial Sequence
  source: /note="Description of Artificial Sequence: Synthetic polypeptide"
EVQLVQSGAEVKKPGESLKISCKGSGYTFTSYNMHWVRQMPGKGLEWMGDIYPGSGDTSYNQKFKGQVTISADKSISTVYLQWSSLKASDTAMYYCARVGGAFPMDYWGQGTTVTVSS

SEQ ID NO: 77 - DNA, 354 bp, Artificial Sequence
  source: /note="Description of Artificial Sequence: Synthetic polynucleotide"
gaagttcaattggtacagtctggcgcagaagtaaagaaaccaggagagagtttgaaaatttcctgcaagggcagtgggtacacattcacgtcctacaatatgcactgggtgagacagatgccaggcaagggcctggagtggatgggagacatatacccaggcagtggagacacaagctataatcagaaattcaaaggacaggtgacgatctccgcagacaaatccatatctacggtctacctccagtggtcctcacttaaagcctccgacaccgccatgtactattgcgctcgggtaggtggcgcgtttccaatggactattggggccaagggaccacagtaaccgtcagctca

SEQ ID NO: 78 - protein, 445 aa, Artificial Sequence
  source: /note="Description of Artificial Sequence: Synthetic polypeptide"
EVQLVQSGAEVKKPGESLKISCKGSGYTFTSYNMHWVRQMPGKGLEWMGDIYPGSGDTSYNQKFKGQVTISADKSISTVYLQWSSLKASDTAMYYCARVGGAFPMDYWGQGTTVTVSSASTKGPSVFPLAPCSRSTSESTAALGCLVKDYFPEPVTVSWNSGALTSGVHTFPAVLQSSGLYSLSSVVTVPSSSLGTKTYTCNVDHKPSNTKVDKRVESKYGPPCPPCPAPEFLGGPSVFLFPPKPKDTLMISRTPEVTCVVVDVSQEDPEVQFNWYVDGVEVHNAKTKPREEQFNSTYRVVSVLTVLHQDWLNGKEYKCKVSNKGLPSSIEKTISKAKGQPREPQVYTLPPSQEEMTKNQVSLTCLVKGFYPSDIAVEWESNGQPENNYKTTPPVLDSDGSFFLYSRLTVDKSRWQEGNVFSCSVMHEALHNHYTQKSLSLSLGK

SEQ ID NO: 79 - DNA, 1335 bp, Artificial Sequence
  source: /note="Description of Artificial Sequence: Synthetic polynucleotide"
gaagttcaattggtacagtctggcgcagaagtaaagaaaccaggagagagtttgaaaatttcctgcaagggcagtgggtacacattcacgtcctacaatatgcactgggtgagacagatgccaggcaagggcctggagtggatgggagacatatacccaggcagtggagacacaagctataatcagaaattcaaaggacaggtgacgatctccgcagacaaatccatatctacggtctacctccagtggtcctcacttaaagcctccgacaccgccatgtactattgcgctcgggtaggtggcgcgtttccaatggactattggggccaagggaccacagtaaccgtcagctcagcctctacaaagggcccctccgtctttccactcgcgccgtgctctcgctccacctcagagtcaactgccgctctgggttgcctggtcaaggactacttcccagagccggtgacagtgagctggaacagtggggccctgacatccggcgttcataccttccccgcagtcctccagtcctcaggcctgtattccctgagcagcgttgtcacagtgccctccagctctcttggcacgaaaacctacacatgcaacgttgatcataagccgtctaataccaaggtggataaaagagtggagagcaagtacggcccaccctgcccgccttgcccagctccggagttcctgggcggaccatccgttttcttgtttccacccaaacctaaagacactctgatgatttcccgaacccctgaagtgacttgcgttgtggtggacgtctcccaggaggacccagaagtgcaattcaactggtacgtggacggggtggaggtgcacaatgcaaaaaccaaaccaagggaggaacagtttaattcaacatatagggttgtgtctgtgctgacggttctgcatcaggactggctgaacggaaaggaatacaagtgcaaggtgtccaacaaaggactgccaagctctatcgagaaaacaatctctaaggccaagggacaacctagagagccccaagtttacaccctgccaccatcacaggaagagatgaccaaaaatcaggtgagcttgacatgcctggtgaagggcttctaccctagcgatattgcggttgagtgggagtcaaatggccagcctgagaacaactataagactactcctcccgtgctggactccgacgggagctttttcctgtattccaggcttacagtcgataagagcagatggcaagaggggaatgtgttttcctgctccgtgatgcacgaggctctccataaccattatactcagaaaagtctctctctgtcactgggcaaa

SEQ ID NO: 80 - protein, 118 aa, Artificial Sequence
  source: /note="Description of Artificial Sequence: Synthetic polypeptide"
EVQLVQSGAEVKKPGESLKISCKGSGYTFTSYNMHWVRQMPGKGLEWMGDIYPGQGDTSYNQKFKGQVTISADKSISTVYLQWSSLKASDTAMYYCARVGGAFPMDYWGQGTTVTVSS

SEQ ID NO: 81 - DNA, 354 bp, Artificial Sequence
  source: /note="Description of Artificial Sequence: Synthetic polynucleotide"
gaagttcaattggtacagtctggcgcagaagtaaagaaaccaggagagagtttgaaaatttcctgcaagggcagtgggtacacattcacgtcctacaatatgcactgggtgagacagatgccaggcaagggcctggagtggatgggagacatatacccaggccagggagacacaagctataatcagaaattcaaaggacaggtgacgatctccgcagacaaatccatatctacggtctacctccagtggtcctcacttaaagcctccgacaccgccatgtactattgcgctcgggtaggtggcgcgtttccaatggactattggggccaagggaccacagtaaccgtcagctca

SEQ ID NO: 82 - protein, 445 aa, Artificial Sequence
  source: /note="Description of Artificial Sequence: Synthetic polypeptide"
EVQLVQSGAEVKKPGESLKISCKGSGYTFTSYNMHWVRQMPGKGLEWMGDIYPGQGDTSYNQKFKGQVTISADKSISTVYLQWSSLKASDTAMYYCARVGGAFPMDYWGQGTTVTVSSASTKGPSVFPLAPCSRSTSESTAALGCLVKDYFPEPVTVSWNSGALTSGVHTFPAVLQSSGLYSLSSVVTVPSSSLGTKTYTCNVDHKPSNTKVDKRVESKYGPPCPPCPAPEFLGGPSVFLFPPKPKDTLMISRTPEVTCVVVDVSQEDPEVQFNWYVDGVEVHNAKTKPREEQFNSTYRVVSVLTVLHQDWLNGKEYKCKVSNKGLPSSIEKTISKAKGQPREPQVYTLPPSQEEMTKNQVSLTCLVKGFYPSDIAVEWESNGQPENNYKTTPPVLDSDGSFFLYSRLTVDKSRWQEGNVFSCSVMHEALHNHYTQKSLSLSLGK

SEQ ID NO: 83 - DNA, 1335 bp, Artificial Sequence
  source: /note="Description of Artificial Sequence: Synthetic polynucleotide"
gaagttcaattggtacagtctggcgcagaagtaaagaaaccaggagagagtttgaaaatttcctgcaagggcagtgggtacacattcacgtcctacaatatgcactgggtgagacagatgccaggcaagggcctggagtggatgggagacatatacccaggccagggagacacaagctataatcagaaattcaaaggacaggtgacgatctccgcagacaaatccatatctacggtctacctccagtggtcctcacttaaagcctccgacaccgccatgtactattgcgctcgggtaggtggcgcgtttccaatggactattggggccaagggaccacagtaaccgtcagctcagcctctacaaagggcccctccgtctttccactcgcgccgtgctctcgctccacctcagagtcaactgccgctctgggttgcctggtcaaggactacttcccagagccggtgacagtgagctggaacagtggggccctgacatccggcgttcataccttccccgcagtcctccagtcctcaggcctgtattccctgagcagcgttgtcacagtgccctccagctctcttggcacgaaaacctacacatgcaacgttgatcataagccgtctaataccaaggtggataaaagagtggagagcaagtacggcccaccctgcccgccttgcccagctccggagttcctgggcggaccatccgttttcttgtttccacccaaacctaaagacactctgatgatttcccgaacccctgaagtgacttgcgttgtggtggacgtctcccaggaggacccagaagtgcaattcaactggtacgtggacggggtggaggtgcacaatgcaaaaaccaaaccaagggaggaacagtttaattcaacatatagggttgtgtctgtgctgacggttctgcatcaggactggctgaacggaaaggaatacaagtgcaaggtgtccaacaaaggactgccaagctctatcgagaaaacaatctctaaggccaagggacaacctagagagccccaagtttacaccctgccaccatcacaggaagagatgaccaaaaatcaggtgagcttgacatgcctggtgaagggcttctaccctagcgatattgcggttgagtgggagtcaaatggccagcctgagaacaactataagactactcctcccgtgctggactccgacgggagctttttcctgtattccaggcttacagtcgataagagcagatggcaagaggggaatgtgttttcctgctccgtgatgcacgaggctctccataaccattatactcagaaaagtctctctctgtcactgggcaaa

SEQ ID NO: 84 - protein, 118 aa, Artificial Sequence; identical to SEQ ID NO: 32
  source: /note="Description of Artificial Sequence: Synthetic polypeptide"

SEQ ID NO: 85 - DNA, 354 bp, Artificial Sequence
  source: /note="Description of Artificial Sequence: Synthetic polynucleotide"
caggtgcaattggtgcagagcggagcagaggtcaaaaagcccggagcaagcgtgaaggtctcatgcaaagcaagcggatacacatttacatcatacaacatgcactgggtcaggcaggctccaggacagggactggagtggatcggggacatctaccctggacagggcgatactagctataatcagaagttcaaaggccgggccaccatgacagctgacaagtctactagtaccgtgtatatggaactgagctccctgcggtctgaagataccgcagtgtactattgcgccagagtcgggggggcatttcctatggattattgggggcaggggactctggtcactgtcagctca

SEQ ID NO: 86 - protein, 448 aa, Artificial Sequence
  source: /note="Description of Artificial Sequence: Synthetic polypeptide"
QVQLVQSGAEVKKPGASVKVSCKASGYTFTSYNMHWVRQAPGQGLEWIGDIYPGQGDTSYNQKFKGRATMTADKSTSTVYMELSSLRSEDTAVYYCARVGGAFPMDYWGQGTLVTVSSASTKGPSVFPLAPSSKSTSGGTAALGCLVKDYFPEPVTVSWNSGALTSGVHTFPAVLQSSGLYSLSSVVTVPSSSLGTQTYICNVNHKPSNTKVDKRVEPKSCDKTHTCPPCPAPELLGGPSVFLFPPKPKDTLMISRTPEVTCVVVAVSHEDPEVKFNWYVDGVEVHNAKTKPREEQYNSTYRVVSVLTVLHQDWLNGKEYKCKVSNKALAAPIEKTISKAKGQPREPQVYTLPPSREEMTKNQVSLTCLVKGFYPSDIAVEWESNGQPENNYKTTPPVLDSDGSFFLYSKLTVDKSRWQQGNVFSCSVMHEALHNHYTQKSLSLSPGK

SEQ ID NO: 87 - DNA, 1344 bp, Artificial Sequence
  source: /note="Description of Artificial Sequence: Synthetic polynucleotide"
caggtgcaattggtgcagagcggagcagaggtcaaaaagcccggagcaagcgtgaaggtctcatgcaaagcaagcggatacacatttacatcatacaacatgcactgggtcaggcaggctccaggacagggactggagtggatcggggacatctaccctggacagggcgatactagctataatcagaagttcaaaggccgggccaccatgacagctgacaagtctactagtaccgtgtatatggaactgagctccctgcggtctgaagataccgcagtgtactattgcgccagagtcgggggggcatttcctatggattattgggggcaggggactctggtcactgtcagctcagctagcaccaagggccccagcgtgttccccctggcccccagcagcaagagcaccagcggcggcacagccgccctgggctgcctggtgaaggactacttccccgagcccgtgaccgtgtcctggaacagcggagccctgacctccggcgtgcacaccttccccgccgtgctgcagagcagcggcctgtacagcctgtccagcgtggtgacagtgcccagcagcagcctgggcacccagacctacatctgcaacgtgaaccacaagcccagcaacaccaaggtggacaagagagtggagcccaagagctgcgacaagacccacacctgccccccctgcccagccccagagctgctgggcggaccctccgtgttcctgttcccccccaagcccaaggacaccctgatgatcagcaggacccccgaggtgacctgcgtggtggtggccgtgagccacgaggacccagaggtgaagttcaactggtacgtggacggcgtggaggtgcacaacgccaagaccaagcccagagaggagcagtacaacagcacctacagggtggtgtccgtgctgaccgtgctgcaccaggactggctgaacggcaaggaatacaagtgcaaggtctccaacaaggccctggcagcccccatcgaaaagaccatcagcaaggccaagggccagccacgggagccccaggtgtacaccctgcccccctcccgggaggagatgaccaagaaccaggtgtccctgacctgtctggtgaagggcttctaccccagcgacatcgccgtggagtgggagagcaacggccagcccgagaacaactacaagaccacccccccagtgctggacagcgacggcagcttcttcctgtacagcaagctgaccgtggacaagtccaggtggcagcagggcaacgtgttcagctgcagcgtgatgcacgaggccctgcacaaccactacacccagaagagcctgagcctgtcccccggcaag

SEQ ID NO: 88 - protein, 111 aa, Artificial Sequence; identical to SEQ ID NO: 20
  source: /note="Description of Artificial Sequence: Synthetic polypeptide"

SEQ ID NO: 89 - DNA, 333 bp, Artificial Sequence
  source: /note="Description of Artificial Sequence: Synthetic polynucleotide"
gacatcgtcctgacacagtctcctgacagcctggcagtgagcctgggcgaaagggcaaccattaattgtagagcttccgagtccgtcgagtactatggcactagtctgatgcagtggtaccagcagaagccagggcagccccctaaactgctgatctatgcagctagcaacgtggagtccggagtcccagaccggttctctggaagtgggtcaggaaccgattttaccctgacaattagctccctgcaggcagaagacgtggccgtctactattgtcagcagagccgcaaggacccaagcacattcggaggggggaccaaagtggaaatcaag

SEQ ID NO: 90 - protein, 218 aa, Artificial Sequence; identical to SEQ ID NO: 22
  source: /note="Description of Artificial Sequence: Synthetic polypeptide"

SEQ ID NO: 91 - DNA, 654 bp, Artificial Sequence
  source: /note="Description of Artificial Sequence: Synthetic polynucleotide"
gacatcgtcctgacacagtctcctgacagcctggcagtgagcctgggcgaaagggcaaccattaattgtagagcttccgagtccgtcgagtactatggcactagtctgatgcagtggtaccagcagaagccagggcagccccctaaactgctgatctatgcagctagcaacgtggagtccggagtcccagaccggttctctggaagtgggtcaggaaccgattttaccctgacaattagctccctgcaggcagaagacgtggccgtctactattgtcagcagagccgcaaggacccaagcacattcggaggggggaccaaagtggaaatcaagcgtacggtggccgctcccagcgtgttcatcttcccccccagcgacgagcagctgaagagcggcaccgccagcgtggtgtgcctgctgaacaacttctacccccgggaggccaaggtgcagtggaaggtggacaacgccctgcagagcggcaacagccaggagagcgtcaccgagcaggacagcaaggactccacctacagcctgagcagcaccctgaccctgagcaaggccgactacgagaagcataaggtgtacgcctgcgaggtgacccaccagggcctgtccagccccgtgaccaagagcttcaacaggggcgagtgc

SEQ ID NO: 92 - protein, 118 aa, Artificial Sequence
  source: /note="Description of Artificial Sequence: Synthetic polypeptide"
QVQLVQSGAEVKKPGASVKVSCKASGYTFTSYNMHWVRQAPGQGLEWMGDIYPGQGDTSYNQKFKGRVTMTRDTSTSTVYMELSSLRSEDTAVYYCARVGGAFPMDYWGQGTTVTVSS

SEQ ID NO: 93 - DNA, 354 bp, Artificial Sequence
  source: /note="Description of Artificial Sequence: Synthetic polynucleotide"
caggtgcagctggtgcagtctggcgccgaagtgaagaaaccaggcgccagcgtgaaggtgtcctgcaaggccagcggctacacctttaccagctacaacatgcactgggtgcgccaggcccctggacagggactggaatggatgggcgacatctaccccggccagggcgacacctcctacaaccagaaattcaagggcagagtgaccatgacccgggacaccagcacctccaccgtgtacatggaactgagcagcctgcggagcgaggacaccgccgtgtactactgtgctagagtgggcggagccttccccatggactattggggccagggcaccaccgtgaccgtgagctca

SEQ ID NO: 94 - protein, 448 aa, Artificial Sequence
  source: /note="Description of Artificial Sequence: Synthetic polypeptide"
QVQLVQSGAEVKKPGASVKVSCKASGYTFTSYNMHWVRQAPGQGLEWMGDIYPGQGDTSYNQKFKGRVTMTRDTSTSTVYMELSSLRSEDTAVYYCARVGGAFPMDYWGQGTTVTVSSASTKGPSVFPLAPSSKSTSGGTAALGCLVKDYFPEPVTVSWNSGALTSGVHTFPAVLQSSGLYSLSSVVTVPSSSLGTQTYICNVNHKPSNTKVDKRVEPKSCDKTHTCPPCPAPELLGGPSVFLFPPKPKDTLMISRTPEVTCVVVAVSHEDPEVKFNWYVDGVEVHNAKTKPREEQYNSTYRVVSVLTVLHQDWLNGKEYKCKVSNKALAAPIEKTISKAKGQPREPQVYTLPPSREEMTKNQVSLTCLVKGFYPSDIAVEWESNGQPENNYKTTPPVLDSDGSFFLYSKLTVDKSRWQQGNVFSCSVMHEALHNHYTQKSLSLSPGK

SEQ ID NO: 95 - DNA, 1344 bp, Artificial Sequence
  source: /note="Description of Artificial Sequence: Synthetic polynucleotide"
caggtgcagctggtgcagtctggcgccgaagtgaagaaaccaggcgccagcgtgaaggtgtcctgcaaggccagcggctacacctttaccagctacaacatgcactgggtgcgccaggcccctggacagggactggaatggatgggcgacatctaccccggccagggcgacacctcctacaaccagaaattcaagggcagagtgaccatgacccgggacaccagcacctccaccgtgtacatggaactgagcagcctgcggagcgaggacaccgccgtgtactactgtgctagagtgggcggagccttccccatggactattggggccagggcaccaccgtgaccgtgagctcagctagcaccaagggccccagcgtgttccccctggcccccagcagcaagagcaccagcggcggcacagccgccctgggctgcctggtgaaggactacttccccgagcccgtgaccgtgtcctggaacagcggagccctgacctccggcgtgcacaccttccccgccgtgctgcagagcagcggcctgtacagcctgtccagcgtggtgacagtgcccagcagcagcctgggcacccagacctacatctgcaacgtgaaccacaagcccagcaacaccaaggtggacaagagagtggagcccaagagctgcgacaagacccacacctgccccccctgcccagccccagagctgctgggcggaccctccgtgttcctgttcccccccaagcccaaggacaccctgatgatcagcaggacccccgaggtgacctgcgtggtggtggccgtgagccacgaggacccagaggtgaagttcaactggtacgtggacggcgtggaggtgcacaacgccaagaccaagcccagagaggagcagtacaacagcacctacagggtggtgtccgtgctgaccgtgctgcaccaggactggctgaacggcaaggaatacaagtgcaaggtctccaacaaggccctggcagcccccatcgaaaagaccatcagcaaggccaagggccagccacgggagccccaggtgtacaccctgcccccctcccgggaggagatgaccaagaaccaggtgtccctgacctgtctggtgaagggcttctaccccagcgacatcgccgtggagtgggagagcaacggccagcccgagaacaactacaagaccacccccccagtgctggacagcgacggcagcttcttcctgtacagcaagctgaccgtggacaagtccaggtggcagcagggcaacgtgttcagctgcagcgtgatgcacgaggccctgcacaaccactacacccagaagagcctgagcctgtcccccggcaag

SEQ ID NO: 96 - protein, 111 aa, Artificial Sequence
  source: /note="Description of Artificial Sequence: Synthetic polypeptide"
AIRLTQSPSSFSASTGDRVTITCRASESVEYYGTSLMQWYQQKPGKAPKLLIYAASNVESGVPSRFSGSGSGTDFTLTISSLQSEDFATYYCQQSRKDPSTFGGGTKVEIK

SEQ ID NO: 97 - DNA, 333 bp, Artificial Sequence
  source: /note="Description of Artificial Sequence: Synthetic polynucleotide"
gccatcagactgacccagagccccagctcctttagcgccagcaccggcgacagagtgaccatcacctgtagagccagcgagagcgtggaatattacggcaccagcctgatgcagtggtatcagcagaagcccggcaaggcccccaagctgctgatctacgccgccagcaatgtggaaagcggcgtgcccagcagattcagcggctctggcagcggcaccgacttcaccctgacaatcagcagcctgcagagcgaggacttcgccacctactactgccagcagagccggaaggaccccagcacatttggcggaggcaccaaggtggaaatcaag

SEQ ID NO: 98 - protein, 218 aa, Artificial Sequence
  source: /note="Description of Artificial Sequence: Synthetic polypeptide"
AIRLTQSPSSFSASTGDRVTITCRASESVEYYGTSLMQWYQQKPGKAPKLLIYAASNVESGVPSRFSGSGSGTDFTLTISSLQSEDFATYYCQQSRKDPSTFGGGTKVEIKRTVAAPSVFIFPPSDEQLKSGTASVVCLLNNFYPREAKVQWKVDNALQSGNSQESVTEQDSKDSTYSLSSTLTLSKADYEKHKVYACEVTHQGLSSPVTKSFNRGEC

SEQ ID NO: 99 - DNA, 654 bp, Artificial Sequence
  source: /note="Description of Artificial Sequence: Synthetic polynucleotide"
gccatcagactgacccagagccccagctcctttagcgccagcaccggcgacagagtgaccatcacctgtagagccagcgagagcgtggaatattacggcaccagcctgatgcagtggtatcagcagaagcccggcaaggcccccaagctgctgatctacgccgccagcaatgtggaaagcggcgtgcccagcagattcagcggctctggcagcggcaccgacttcaccctgacaatcagcagcctgcagagcgaggacttcgccacctactactgccagcagagccggaaggaccccagcacatttggcggaggcaccaaggtggaaatcaagcgtacggtggccgctcccagcgtgttcatcttcccccccagcgacgagcagctgaagagcggcaccgccagcgtggtgtgcctgctgaacaacttctacccccgggaggccaaggtgcagtggaaggtggacaacgccctgcagagcggcaacagccaggagagcgtcaccgagcaggacagcaaggactccacctacagcctgagcagcaccctgaccctgagcaaggccgactacgagaagcataaggtgtacgcctgcgaggtgacccaccagggcctgtccagccccgtgaccaagagcttcaacaggggcgagtgc

SEQ ID NO: 100 - protein, 118 aa, Artificial Sequence
  source: /note="Description of Artificial Sequence: Synthetic polypeptide"
QVQLVQSGAEVKKPGESLKISCKGSGYTFTSYNMHWVRQMPGKGLEWMGDIYPGNGDTSYNQKFKGQVTISADKSISTVYLQWSSLKASDTAMYYCARVGGAFPMDYWGQGTTVTVSS

SEQ ID NO: 101 - DNA, 354 bp, Artificial Sequence
  source: /note="Description of Artificial Sequence: Synthetic polynucleotide"
caggtgcaattggtacagtctggcgcagaagtaaagaaaccaggagagagtttgaaaatttcctgcaagggcagtgggtacacattcacgtcctacaatatgcactgggtgagacagatgccaggcaagggcctggagtggatgggagacatatacccaggcaatggagacacaagctataatcagaaattcaaaggacaggtgacgatctccgcagacaaatccatatctacggtctacctccagtggtcctcacttaaagcctccgacaccgccatgtactattgcgctcgggtaggtggcgcgtttccaatggactattggggccaagggaccacagtaaccgtcagctca

SEQ ID NO: 102 - protein, 448 aa, Artificial Sequence
  source: /note="Description of Artificial Sequence: Synthetic polypeptide"
QVQLVQSGAEVKKPGESLKISCKGSGYTFTSYNMHWVRQMPGKGLEWMGDIYPGNGDTSYNQKFKGQVTISADKSISTVYLQWSSLKASDTAMYYCARVGGAFPMDYWGQGTTVTVSSASTKGPSVFPLAPSSKSTSGGTAALGCLVKDYFPEPVTVSWNSGALTSGVHTFPAVLQSSGLYSLSSVVTVPSSSLGTQTYICNVNHKPSNTKVDKRVEPKSCDKTHTCPPCPAPELLGGPSVFLFPPKPKDTLMISRTPEVTCVVVAVSHEDPEVKFNWYVDGVEVHNAKTKPREEQYNSTYRVVSVLTVLHQDWLNGKEYKCKVSNKALAAPIEKTISKAKGQPREPQVYTLPPSREEMTKNQVSLTCLVKGFYPSDIAVEWESNGQPENNYKTTPPVLDSDGSFFLYSKLTVDKSRWQQGNVFSCSVMHEALHNHYTQKSLSLSPGK

SEQ ID NO: 103 - DNA, 1344 bp, Artificial Sequence
  source: /note="Description of Artificial Sequence: Synthetic polynucleotide"
caggtgcaattggtacagtctggcgcagaagtaaagaaaccaggagagagtttgaaaatttcctgcaagggcagtgggtacacattcacgtcctacaatatgcactgggtgagacagatgccaggcaagggcctggagtggatgggagacatatacccaggcaatggagacacaagctataatcagaaattcaaaggacaggtgacgatctccgcagacaaatccatatctacggtctacctccagtggtcctcacttaaagcctccgacaccgccatgtactattgcgctcgggtaggtggcgcgtttccaatggactattggggccaagggaccacagtaaccgtcagctcagctagcaccaagggccccagcgtgttccccctggcccccagcagcaagagcaccagcggcggcacagccgccctgggctgcctggtgaaggactacttccccgagcccgtgaccgtgtcctggaacagcggagccctgacctccggcgtgcacaccttccccgccgtgctgcagagcagcggcctgtacagcctgtccagcgtggtgacagtgcccagcagcagcctgggcacccagacctacatctgcaacgtgaaccacaagcccagcaacaccaaggtggacaagagagtggagcccaagagctgcgacaagacccacacctgccccccctgcccagccccagagctgctgggcggaccctccgtgttcctgttcccccccaagcccaaggacaccctgatgatcagcaggacccccgaggtgacctgcgtggtggtggccgtgagccacgaggacccagaggtgaagttcaactggtacgtggacggcgtggaggtgcacaacgccaagaccaagcccagagaggagcagtacaacagcacctacagggtggtgtccgtgctgaccgtgctgcaccaggactggctgaacggcaaggaatacaagtgcaaggtctccaacaaggccctggcagcccccatcgaaaagaccatcagcaaggccaagggccagccacgggagccccaggtgtacaccctgcccccctcccgggaggagatgaccaagaaccaggtgtccctgacctgtctggtgaagggcttctaccccagcgacatcgccgtggagtgggagagcaacggccagcccgagaacaactacaagaccacccccccagtgctggacagcgacggcagcttcttcctgtacagcaagctgaccgtggacaagtccaggtggcagcagggcaacgtgttcagctgcagcgtgatgcacgaggccctgcacaaccactacacccagaagagcctgagcctgtcccccggcaag

SEQ ID NO: 104 - protein, 111 aa, Artificial Sequence; identical to SEQ ID NO: 64
  source: /note="Description of Artificial Sequence: Synthetic polypeptide"

SEQ ID NO: 105 - DNA, 333 bp, Artificial Sequence
  source: /note="Description of Artificial Sequence: Synthetic polynucleotide"
gcaatacagttgacacagagtccttcaagtttgtccgcttccgttggcgaccgagtgacaatcacctgtagagcatccgagtcagtggagtattatggcactagcctgatgcagtggtatcagcaaaagccagggaaagccccaaagctgctgatatatgccgcgagtaacgtcgagtcaggggtgccatcaagattctccggttccgggtccggaaccgacttcacactgaccatctcttcccttcagccagaggacttcgctacgtacttttgccagcagtcacggaaagatccctctactttcggaggtgggacaaaagtcgaaattaaa

SEQ ID NO: 106 - protein, 218 aa, Artificial Sequence; identical to SEQ ID NO: 66
  source: /note="Description of Artificial Sequence: Synthetic polypeptide"

SEQ ID NO: 107 - DNA, 654 bp, Artificial Sequence
  source: /note="Description of Artificial Sequence: Synthetic polynucleotide"
gcaatacagttgacacagagtccttcaagtttgtccgcttccgttggcgaccgagtgacaatcacctgtagagcatccgagtcagtggagtattatggcactagcctgatgcagtggtatcagcaaaagccagggaaagccccaaagctgctgatatatgccgcgagtaacgtcgagtcaggggtgccatcaagattctccggttccgggtccggaaccgacttcacactgaccatctcttcccttcagccagaggacttcgctacgtacttttgccagcagtcacggaaagatccctctactttcggaggtgggacaaaagtcgaaattaaacgtacggtggccgctcccagcgtgttcatcttcccccccagcgacgagcagctgaagagcggcaccgccagcgtggtgtgcctgctgaacaacttctacccccgggaggccaaggtgcagtggaaggtggacaacgccctgcagagcggcaacagccaggagagcgtcaccgagcaggacagcaaggactccacctacagcctgagcagcaccctgaccctgagcaaggccgactacgagaagcataaggtgtacgcctgcgaggtgacccaccagggcctgtccagccccgtgaccaagagcttcaacaggggcgagtgc

SEQ ID NO: 108 - protein, 327 aa, Homo sapiens
ASTKGPSVFPLAPCSRSTSESTAALGCLVKDYFPEPVTVSWNSGALTSGVHTFPAVLQSSGLYSLSSVVTVPSSSLGTKTYTCNVDHKPSNTKVDKRVESKYGPPCPPCPAPEFLGGPSVFLFPPKPKDTLMISRTPEVTCVVVDVSQEDPEVQFNWYVDGVEVHNAKTKPREEQFNSTYRVVSVLTVLHQDWLNGKEYKCKVSNKGLPSSIEKTISKAKGQPREPQVYTLPPSQEEMTKNQVSLTCLVKGFYPSDIAVEWESNGQPENNYKTTPPVLDSDGSFFLYSRLTVDKSRWQEGNVFSCSVMHEALHNHYTQKSLSLSLGK

SEQ ID NO: 109 - protein, 107 aa, Homo sapiens [sequence omitted]

SEQ ID NO: 110 - protein, 326 aa, Homo sapiens
ASTKGPSVFPLAPCSRSTSESTAALGCLVKDYFPEPVTVSWNSGALTSGVHTFPAVLQSSGLYSLSSVVTVPSSSLGTKTYTCNVDHKPSNTKVDKRVESKYGPPCPPCPAPEFLGGPSVFLFPPKPKDTLMISRTPEVTCVVVDVSQEDPEVQFNWYVDGVEVHNAKTKPREEQFNSTYRVVSVLTVLHQDWLNGKEYKCKVSNKGLPSSIEKTISKAKGQPREPQVYTLPPSQEEMTKNQVSLTCLVKGFYPSDIAVEWESNGQPENNYKTTPPVLDSDGSFFLYSRLTVDKSRWQEGNVFSCSVMHEALHNHYTQKSLSLSLG

SEQ ID NO: 111 - protein, 330 aa, Homo sapiens
ASTKGPSVFPLAPSSKSTSGGTAALGCLVKDYFPEPVTVSWNSGALTSGVHTFPAVLQSSGLYSLSSVVTVPSSSLGTQTYICNVNHKPSNTKVDKRVEPKSCDKTHTCPPCPAPELLGGPSVFLFPPKPKDTLMISRTPEVTCVVVDVSHEDPEVKFNWYVDGVEVHNAKTKPREEQYNSTYRVVSVLTVLHQDWLNGKEYKCKVSNKALPAPIEKTISKAKGQPREPQVYTLPPSREEMTKNQVSLTCLVKGFYPSDIAVEWESNGQPENNYKTTPPVLDSDGSFFLYSKLTVDKSRWQQGNVFSCSVMHEALHNHYTQKSLSLSPGK

SEQ ID NO: 112 - protein, 330 aa, Homo sapiens
ASTKGPSVFPLAPSSKSTSGGTAALGCLVKDYFPEPVTVSWNSGALTSGVHTFPAVLQSSGLYSLSSVVTVPSSSLGTQTYICNVNHKPSNTKVDKRVEPKSCDKTHTCPPCPAPELLGGPSVFLFPPKPKDTLMISRTPEVTCVVVDVSHEDPEVKFNWYVDGVEVHNAKTKPREEQYASTYRVVSVLTVLHQDWLNGKEYKCKVSNKALPAPIEKTISKAKGQPREPQVYTLPPSREEMTKNQVSLTCLVKGFYPSDIAVEWESNGQPENNYKTTPPVLDSDGSFFLYSKLTVDKSRWQQGNVFSCSVMHEALHNHYTQKSLSLSPGK

SEQ ID NO: 113 - protein, 330 aa, Homo sapiens
ASTKGPSVFPLAPSSKSTSGGTAALGCLVKDYFPEPVTVSWNSGALTSGVHTFPAVLQSSGLYSLSSVVTVPSSSLGTQTYICNVNHKPSNTKVDKRVEPKSCDKTHTCPPCPAPELLGGPSVFLFPPKPKDTLMISRTPEVTCVVVAVSHEDPEVKFNWYVDGVEVHNAKTKPREEQYNSTYRVVSVLTVLHQDWLNGKEYKCKVSNKALAAPIEKTISKAKGQPREPQVYTLPPSREEMTKNQVSLTCLVKGFYPSDIAVEWESNGQPENNYKTTPPVLDSDGSFFLYSKLTVDKSRWQQGNVFSCSVMHEALHNHYTQKSLSLSPGK

SEQ ID NO: 114 - protein, 330 aa, Homo sapiens
ASTKGPSVFPLAPSSKSTSGGTAALGCLVKDYFPEPVTVSWNSGALTSGVHTFPAVLQSSGLYSLSSVVTVPSSSLGTQTYICNVNHKPSNTKVDKRVEPKSCDKTHTCPPCPAPEAAGGPSVFLFPPKPKDTLMISRTPEVTCVVVDVSHEDPEVKFNWYVDGVEVHNAKTKPREEQYNSTYRVVSVLTVLHQDWLNGKEYKCKVSNKALPAPIEKTISKAKGQPREPQVYTLPPSREEMTKNQVSLTCLVKGFYPSDIAVEWESNGQPENNYKTTPPVLDSDGSFFLYSKLTVDKSRWQQGNVFSCSVMHEALHNHYTQKSLSLSPGK

SEQ ID NO: 115 - DNA, 354 bp, Artificial Sequence
  source: /note="Description of Artificial Sequence: Synthetic polynucleotide"
caggtccagctggtccagagcggagcagaggtcaaaaagcccggagcaagcgtgaaggtctcatgcaaagcaagcggatacacatttacatcatacaacatgcactggatcaggcaggctccaggacagggactggagtggatcggggacatctaccctggaaacggcgatactagctataatcagaagttcaaaggccgggccaccctgacagctgacaagtctactagtaccgtgtatatggagctgagctccctgcggtctgaagataccgcagtgtactattgcgccagagtcgggggggcatttcctatggattattgggggcaggggactctggtcactgtctcctcc

SEQ ID NO: 116 - protein, 445 aa, Artificial Sequence
  source: /note="Description of Artificial Sequence: Synthetic polypeptide"
QVQLVQSGAEVKKPGASVKVSCKASGYTFTSYNMHWIRQAPGQGLEWIGDIYPGNGDTSYNQKFKGRATLTADKSTSTVYMELSSLRSEDTAVYYCARVGGAFPMDYWGQGTLVTVSSASTKGPSVFPLAPCSRSTSESTAALGCLVKDYFPEPVTVSWNSGALTSGVHTFPAVLQSSGLYSLSSVVTVPSSSLGTKTYTCNVDHKPSNTKVDKRVESKYGPPCPPCPAPEFLGGPSVFLFPPKPKDTLMISRTPEVTCVVVDVSQEDPEVQFNWYVDGVEVHNAKTKPREEQFNSTYRVVSVLTVLHQDWLNGKEYKCKVSNKGLPSSIEKTISKAKGQPREPQVYTLPPSQEEMTKNQVSLTCLVKGFYPSDIAVEWESNGQPENNYKTTPPVLDSDGSFFLYSRLTVDKSRWQEGNVFSCSVMHEALHNHYTQKSLSLSLGK

SEQ ID NO: 117 - DNA, 1335 bp, Artificial Sequence
  source: /note="Description of Artificial Sequence: Synthetic polynucleotide"
caggtccagctggtccagagcggagcagaggtcaaaaagcccggagcaagcgtgaaggtctcatgcaaagcaagcggatacacatttacatcatacaacatgcactggatcaggcaggctccaggacagggactggagtggatcggggacatctaccctggaaacggcgatactagctataatcagaagttcaaaggccgggccaccctgacagctgacaagtctactagtaccgtgtatatggagctgagctccctgcggtctgaagataccgcagtgtactattgcgccagagtcgggggggcatttcctatggattattgggggcaggggactctggtcactgtctcctccgctagcaccaagggcccatccgtcttccccctggcgccctgctccaggagcacctccgagagcacagccgccctgggctgcctggtcaaggactacttccccgaaccggtgacggtgtcgtggaactcaggcgccctgaccagcggcgtgcacaccttcccggctgtcctacagtcctcaggactctactccctcagcagcgtggtgaccgtgccctccagcagcttgggcacgaagacctacacctgcaacgtagatcacaagcccagcaacaccaaggtggacaagagagttgagtccaaatatggtcccccatgcccaccatgcccagcacctgagttcctggggggaccatcagtcttcctgttccccccaaaacccaaggacactctcatgatctcccggacccctgaggtcacgtgcgtggtggtggacgtgagccaggaagaccccgaggtccagttcaactggtacgtggatggcgtggaggtgcataatgccaagacaaagccgcgggaggagcagttcaacagcacgtaccgtgtggtcagcgtcctcaccgtcctgcaccaggactggctgaacggcaaggagtacaagtgcaaggtctccaacaaaggcctcccgtcctccatcgagaaaaccatctccaaagccaaagggcagccccgagagccacaggtgtacaccctgcccccatcccaggaggagatgaccaagaaccaggtcagcctgacctgcctggtcaaaggcttctaccccagcgacatcgccgtggagtgggagagcaatgggcagccggagaacaactacaagaccacgcctcccgtgctggactccgacggctccttcttcctctacagcaggctaaccgtggacaagagcaggtggcaggaggggaatgtcttctcatgctccgtgatgcatgaggctctgcacaaccactacacacagaagagcctctccctgtctctgggtaaa

SEQ ID NO: 118 - DNA, 333 bp, Artificial Sequence; identical to SEQ ID NO: 89
  source: /note="Description of Artificial Sequence: Synthetic polynucleotide"

SEQ ID NO: 119 - DNA, 654 bp, Artificial Sequence
  source: /note="Description of Artificial Sequence: Synthetic polynucleotide"
gacatcgtcctgacacagtctcctgacagcctggcagtgagcctgggcgaaagggcaaccattaattgtagagcttccgagtccgtcgagtactatggcactagtctgatgcagtggtaccagcagaagccagggcagccccctaaactgctgatctatgcagctagcaacgtggagtccggagtcccagaccggttctctggaagtgggtcaggaaccgattttaccctgacaattagctccctgcaggcagaagacgtggccgtctactattgtcagcagagccgcaaggacccaagcacattcggaggggggaccaaagtggaaatcaagcggactgttgctgcaccatctgtcttcatcttcccgccatctgatgagcagttgaaatctggaactgcctctgttgtgtgcctgctgaataacttctatcccagagaggccaaagtacagtggaaggtggataacgccctccaatcgggtaactcccaggagagtgtcacagagcaggacagcaaggacagcacctacagcctcagcagcaccctgacgctgagcaaagcagactacgagaaacacaaagtctacgcctgcgaagtcacccatcagggcctgagttcaccggtgacaaagagcttcaacaggggagagtgt

SEQ ID NO: 120 - DNA, 354 bp, Artificial Sequence
  source: /note="Description of Artificial Sequence: Synthetic polynucleotide"
caggtccagctggtccagagcggagcagaggtcaaaaagcccggagcaagcgtgaaggtctcatgcaaagcaagcggatacacatttacatcatacaacatgcactgggtcaggcaggctccaggacagggactggagtggatcggggacatctaccctggaaacggcgatactagctataatcagaagttcaaaggccgggccaccatgacagctgacaagtctactagtaccgtgtatatggagctgagctccctgcggtctgaagataccgcagtgtactattgcgccagagtcgggggggcatttcctatggattattgggggcaggggactctggtcactgtctcctcc

SEQ ID NO: 121 - protein, 445 aa, Artificial Sequence
  source: /note="Description of Artificial Sequence: Synthetic polypeptide"
QVQLVQSGAEVKKPGASVKVSCKASGYTFTSYNMHWVRQAPGQGLEWIGDIYPGNGDTSYNQKFKGRATMTADKSTSTVYMELSSLRSEDTAVYYCARVGGAFPMDYWGQGTLVTVSSASTKGPSVFPLAPCSRSTSESTAALGCLVKDYFPEPVTVSWNSGALTSGVHTFPAVLQSSGLYSLSSVVTVPSSSLGTKTYTCNVDHKPSNTKVDKRVESKYGPPCPPCPAPEFLGGPSVFLFPPKPKDTLMISRTPEVTCVVVDVSQEDPEVQFNWYVDGVEVHNAKTKPREEQFNSTYRVVSVLTVLHQDWLNGKEYKCKVSNKGLPSSIEKTISKAKGQPREPQVYTLPPSQEEMTKNQVSLTCLVKGFYPSDIAVEWESNGQPENNYKTTPPVLDSDGSFFLYSRLTVDKSRWQEGNVFSCSVMHEALHNHYTQKSLSLSLGK

SEQ ID NO: 122 - DNA, 1335 bp, Artificial Sequence
  source: /note="Description of Artificial Sequence: Synthetic polynucleotide"
caggtccagctggtccagagcggagcagaggtcaaaaagcccggagcaagcgtgaaggtctcatgcaaagcaagcggatacacatttacatcatacaacatgcactgggtcaggcaggctccaggacagggactggagtggatcggggacatctaccctggaaacggcgatactagctataatcagaagttcaaaggccgggccaccatgacagctgacaagtctactagtaccgtgtatatggagctgagctccctgcggtctgaagataccgcagtgtactattgcgccagagtcgggggggcatttcctatggattattgggggcaggggactctggtcactgtctcctccgctagcaccaagggcccatccgtcttccccctggcgccctgctccaggagcacctccgagagcacagccgccctgggctgcctggtcaaggactacttccccgaaccggtgacggtgtcgtggaactcaggcgccctgaccagcggcgtgcacaccttcccggctgtcctacagtcctcaggactctactccctcagcagcgtggtgaccgtgccctccagcagcttgggcacgaagacctacacctgcaacgtagatcacaagcccagcaacaccaaggtggacaagagagttgagtccaaatatggtcccccatgcccaccatgcccagcacctgagttcctggggggaccatcagtcttcctgttccccccaaaacccaaggacactctcatgatctcccggacccctgaggtcacgtgcgtggtggtggacgtgagccaggaagaccccgaggtccagttcaactggtacgtggatggcgtggaggtgcataatgccaagacaaagccgcgggaggagcagttcaacagcacgtaccgtgtggtcagcgtcctcaccgtcctgcaccaggactggctgaacggcaaggagtacaagtgcaaggtctccaacaaaggcctcccgtcctccatcgagaaaaccatctccaaagccaaagggcagccccgagagccacaggtgtacaccctgcccccatcccaggaggagatgaccaagaaccaggtcagcctgacctgcctggtcaaaggcttctaccccagcgacatcgccgtggagtgggagagcaatgggcagccggagaacaactacaagaccacgcctcccgtgctggactccgacggctccttcttcctctacagcaggctaaccgtggacaagagcaggtggcaggaggggaatgtcttctcatgctccgtgatgcatgaggctctgcacaaccactacacacagaagagcctctccctgtctctgggtaaa

SEQ ID NO: 123 - DNA, 333 bp, Artificial Sequence
  source: /note="Description of Artificial Sequence: Synthetic polynucleotide"
gacatcgtcctgacacagtctcctgacagcctggcagtgagcctgggcgaaagggcaaccattaattgtagagcttccgagtccgtcgagtactatggcactagtctgatgcagtggtaccagcagaagccagggcagccccctaaactgctgatctatgcagctagcaacgtggagtccggagtcccagaccggttctctggaagtgggtcaggaaccgattttaccctgacaattagctccctgcaggcagaagacgtggccgtctacttttgtcagcagagccgcaaggacccaagcacattcggaggggggaccaaagtggaaatcaag

SEQ ID NO: 124 - DNA, 654 bp, Artificial Sequence
  source: /note="Description of Artificial Sequence: Synthetic polynucleotide"
gacatcgtcctgacacagtctcctgacagcctggcagtgagcctgggcgaaagggcaaccattaattgtagagcttccgagtccgtcgagtactatggcactagtctgatgcagtggtaccagcagaagccagggcagccccctaaactgctgatctatgcagctagcaacgtggagtccggagtcccagaccggttctctggaagtgggtcaggaaccgattttaccctgacaattagctccctgcaggcagaagacgtggccgtctacttttgtcagcagagccgcaaggacccaagcacattcggaggggggaccaaagtggaaatcaagcggactgttgctgcaccatctgtcttcatcttcccgccatctgatgagcagttgaaatctggaactgcctctgttgtgtgcctgctgaataacttctatcccagagaggccaaagtacagtggaaggtggataacgccctccaatcgggtaactcccaggagagtgtcacagagcaggacagcaaggacagcacctacagcctcagcagcaccctgacgctgagcaaagcagactacgagaaacacaaagtctacgcctgcgaagtcacccatcagggcctgagttcaccggtgacaaagagcttcaacaggggagagtgt

SEQ ID NO: 125 - DNA, 333 bp, Artificial Sequence; identical to SEQ ID NO: 105
  source: /note="Description of Artificial Sequence: Synthetic polynucleotide"

SEQ ID NO: 126 - DNA, 654 bp, Artificial Sequence
  source: /note="Description of Artificial Sequence: Synthetic polynucleotide"
gcaatacagttgacacagagtccttcaagtttgtccgcttccgttggcgaccgagtgacaatcacctgtagagcatccgagtcagtggagtattatggcactagcctgatgcagtggtatcagcaaaagccagggaaagccccaaagctgctgatatatgccgcgagtaacgtcgagtcaggggtgccatcaagattctccggttccgggtccggaaccgacttcacactgaccatctcttcccttcagccagaggacttcgctacgtacttttgccagcagtcacggaaagatccctctactttcggaggtgggacaaaagtcgaaattaaacgtacggtggcagctccgtctgttttcatctttccacctagcgacgagcaactcaaaagtggtacagcatccgtggtttgtctgctgaacaatttttaccccagggaggctaaggtccagtggaaagtcgataacgctcttcagtctggcaacagtcaggagagcgtcacagagcaggactctaaggatagcacttatagtctgtcctccacgctgacactgtctaaagcggattatgagaagcacaaggtttacgcctgtgaggtaacgcaccaaggactctcctccccagttaccaaatctttcaacagaggagaatgt

SEQ ID NO: 127 - DNA, 333 bp, Artificial Sequence
  source: /note="Description of Artificial Sequence: Synthetic polynucleotide"
gagattgttcttacgcaaagtcccgccacacttagtttgtcaccaggagagcgcgccaccctgagctgcagagcttcagagagtgtggaatactacggcacatccctgatgcagtggtatcagcagaaaccaggacaggctcctcggctgctgatctacgcagccagcaacgtcgagtccggcattccagccagattttctgggtcaggatctggaactgactttacactgacaatctccagcctggaacccgaggacattgctgtgtatttttgtcaacagtcccggaaggaccccagtacctttggaggtggaaccaaggtagagataaag

SEQ ID NO: 128 - DNA, 654 bp, Artificial Sequence
  source: /note="Description of Artificial Sequence: Synthetic polynucleotide"
gagattgttcttacgcaaagtcccgccacacttagtttgtcaccaggagagcgcgccaccctgagctgcagagcttcagagagtgtggaatactacggcacatccctgatgcagtggtatcagcagaaaccaggacaggctcctcggctgctgatctacgcagccagcaacgtcgagtccggcattccagccagattttctgggtcaggatctggaactgactttacactgacaatctccagcctggaacccgaggacattgctgtgtatttttgtcaacagtcccggaaggaccccagtacctttggaggtggaaccaaggtagagataaagcgtacggtggcagctccgtctgttttcatctttccacctagcgacgagcaactcaaaagtggtacagcatccgtggtttgtctgctgaacaatttttaccccagggaggctaaggtccagtggaaagtcgataacgctcttcagtctggcaacagtcaggagagcgtcacagagcaggactctaaggatagcacttatagtctgtcctccacgctgacactgtctaaagcggattatgagaagcacaaggtttacgcctgtgaggtaacgcaccaaggactctcctccccagttaccaaatctttcaacagaggagaatgt

SEQ ID NO: 129 - protein, 301 aa, Homo sapiens
MFSHLPFDCVLLLLLLLLTRSSEVEYRAEVGQNAYLPCFYTPAAPGNLVPVCWGKGACPVFECGNVVLRTDERDVNYWTSRYWLNGDFRKGDVSLTIENVTLADSGIYCCRIQIPGIMNDEKFNLKLVIKPAKVTPAPTRQRDFTAAFPRMLTTRGHGPAETQTLGSLPDINLTQISTLANELRDSRLANDLRDSGATIRIGIYIGAGICAGLALALIFGALIFKWYSHSKEKIQNLSLISLANLPPSGLANAVAEGIRSEENIYTIEENVYEVEEPNEYYCYVSSRQQPSQPLGCRFAMP

SEQ ID NO: 130 - protein, 135 aa, Homo sapiens
METDTLLLWVLLLWVPGSTGSEVEYRAEVGQNAYLPCFYTPAAPGNLVPVCWGKGACPVFECGNVVLRTDERDVNYWTSRYWLNGDFRKGDVSLTIENVTLADSGIYCCRIQIPGIMNDEKFNLKLVIKHHHHHH

SEQ ID NO: 131 - protein, 225 aa, Artificial Sequence
  source: /note="Description of Artificial Sequence: Synthetic polypeptide"
QVQLVQSGAEVKKPGASVKVSCKASGYTFTSYNMHWVRQAPGQGLEWIGDIYPGQGDTSYNQKFKGRATMTADKSTSTVYMELSSLRSEDTAVYYCARVGGAFPMDYWGQGTLVTVSSASTKGPSVFPLAPSSKSTSGGTAALGCLVKDYFPEPVTVSWNSGALTSGVHTFPAVLQSSGLYSLSSVVTVPSSSLGTQTYICNVNHKPSNTKVDKRVEPKSCDKTH

SEQ ID NO: 132 - protein, 218 aa, Artificial Sequence; identical to SEQ ID NO: 22
  source: /note="Description of Artificial Sequence: Synthetic polypeptide"

SEQ ID NO: 133 - protein, 6 aa, Artificial Sequence
  source: /note="Description of Artificial Sequence: Synthetic 6xHis tag"
HHHHHH

SEQ ID NO: 134 - protein, 98 aa, Artificial Sequence
  source: /note="Description of Artificial Sequence: Synthetic polypeptide"
QAYLQQSGAELVRPGASVKMSCKASGYTFTSYNMHWVKQTPRQGLEWIGAIYPGNGDTSYNQKFKGKATLTVDKSSSTAYMQLSSLTSEDSAVYFCAR

SEQ ID NO: 135 - protein, 111 aa, Artificial Sequence
  source: /note="Description of Artificial Sequence: Synthetic polypeptide"
DIVLTQSPASLAVSLGQRATISCRASESVEYYGTSLMQWYQQKPGQPPKLLIYAASNVESGVPARFSGSGSGTDFSLNIHPVEEDDIAMYFCQQSRKVPSTFGGGTKLEIK

SEQ ID NO: 136 - protein, 6 aa, Artificial Sequence
  source: /note="Description of Artificial Sequence: Synthetic peptide"
GACPVF

SEQ ID NO: 137 - protein, 9 aa, Artificial Sequence
  source: /note="Description of Artificial Sequence: Synthetic peptide"
NDEKFNLKL

SEQ ID NO: 138 - protein, 4 aa, Artificial Sequence
  source: /note="Description of Artificial Sequence: Synthetic peptide"
IMND

SEQ ID NO: 139 - protein, 114 aa, Homo sapiens
SEVEYRAEVGQNAYLPCFYTPAAPGNLVPVCWGKGACPVFECGNVVLRTDERDVNYWTSRYWLNGDFRKGDVSLTIENVTLADSGIYCCRIQIPGIMNDEKFNLKLVIKPAKVT

SEQ ID NO: 140 - protein, 21 aa, Homo sapiens
TPAAPGNLVPVCWGKGACPVF

SEQ ID NO: 141 - protein, 5 aa, Homo sapiens
RDVNY

SEQ ID NO: 142 - protein, 7 aa, Homo sapiens
EKFNLKL